European Patent Application EP 4 759 827 A2, published June 17, 2026. Title: NUCLEIC ACID VACCINE AGAINST THE SARS-CoV-2 CORONAVIRUS. Applicant: INSTITUT PASTEUR. The sequence listing filed with the application follows.

SEQUENCE LISTING (66 sequences)

SEQ ID NO: 1 - DNA, 3822 bp, synthetic construct
  misc_feature 1..3822: note = synthetic polynucleotide for Antigen_1_nCov_Spike_full_opt_h.sapiens
  source 1..3822: mol_type = other DNA
  CDS 1..3822
atgttcgtgtttctggtgctgctgcctctggtgtccagccagtgtgtgaacctgaccaccagaacacagctgcctccagcctacaccaacagctttaccagaggcgtgtactaccccgacaaggtgttcagatccagcgtgctgcactctacccaggacctgttcctgcctttcttcagcaacgtgacctggttccacgccatccacgtgtccggcaccaatggcaccaagagattcgacaaccccgtgctgcccttcaacgacggggtgtactttgccagcaccgagaagtccaacatcatcagaggctggatcttcggcaccacactggacagcaagacccagagcctgctgatcgtgaacaacgccaccaacgtggtcatcaaagtgtgcgagttccagttctgcaacgaccccttcctgggcgtctactaccacaagaacaacaagagctggatggaaagcgagttccgggtgtacagcagcgccaacaactgcaccttcgagtacgtgtcccagcctttcctgatggacctggaaggcaagcagggcaacttcaagaacctgcgcgagttcgtgttcaagaacatcgacggctacttcaagatctacagcaagcacacccctatcaacctcgtgcgggatctgcctcagggcttctctgctctggaacccctggtggatctgcccatcggcatcaacatcacccggtttcagacactgctggccctgcacagaagctacctgacacctggcgatagcagcagcggatggacagctggtgccgccgcttactatgtgggctacctgcagcctagaaccttcctgctgaagtacaacgagaacggcaccatcaccgacgccgtggattgtgctctggatcctctgagcgagacaaagtgcaccctgaagtccttcaccgtggaaaagggcatctaccagaccagcaacttccgggtgcagcccaccgaatccatcgtgcggttccccaatatcaccaatctgtgccccttcggcgaggtgttcaatgccaccagattcgcctctgtgtacgcctggaaccggaagcggatcagcaattgcgtggccgactactccgtgctgtacaactccgccagcttcagcaccttcaagtgctacggcgtgtcccctaccaagctgaacgacctgtgcttcacaaacgtgtacgccgacagcttcgtgatccggggagatgaagtgcggcagattgcccctggacagacaggcaagatcgccgactacaactacaagctgcccgacgacttcaccggctgtgtgattgcctggaacagcaacaacctggactccaaagtcggcggcaactacaattacctgtaccggctgttccggaagtccaatctgaagcccttcgagcgggacatctccaccgagatctatcaggccggcagcaccccttgtaacggcgtggaaggcttcaactgctacttcccactgcagtcctacggctttcagcccacaaatggcgtgggctatcagccctacagagtggtggtgctgagcttcgaactgctgcatgcccctgccacagtgtgcggccctaagaaaagcaccaatctcgtgaagaacaaatgcgtgaacttcaacttcaacggcctgaccggcaccggcgtgctgacagagagcaacaagaagttcctgccattccagcagtttggccgggatatcgccgataccacagacgccgttagagatccccagacactggaaatcctggacatcaccccttgcagcttcggcggagtgtctgtgatcacccctggcaccaacaccagcaatcaggtggcagtgctgtaccaggacgtgaactgtaccgaagtgcccgtggccattcacgccgatcagctgacacctacatggcgggtgtactccaccggcagcaatgtgtttcagaccagagccggctgtctgatcggagccgagcacgtgaacaatagctacgagtgcgacatccccatcggcgctggcatctgtgccagctaccagacacagacaaacagccccagacgggccagatctgtggccagccagagcatcattgcctacacaatgtctctgggcgccgagaacagcgtggcctactccaacaactctatcgctatccccaccaacttcaccatcagcgtgaccacagagatcctgcctgtgtccatgaccaagaccagcgtggactgcaccatgtacatctgcggcgattccaccgagtgctccaacctgctgctgcagtacggcagcttctgcacccagctgaatagagccctgacagggatcgccgtggaacaggacaagaacacccaagaggtgttcgcccaagtgaagcagatctacaagacccctcctatcaaggacttcggcggcttcaatttcagccagattctgcccgatcctagcaagcccagcaagcggagcttcatcgaggacctgctgttcaacaaagtgacactggccgacgccggcttcatcaagcagtatggcgattgtctgggcgacattgccgccagggatctgatttgcgcccagaagtttaacggactgacagtgctgcctcctctgctgaccgatgagatgatcgcccagtacacatctgccctgctggccggcacaatcacaagcggctggacatttggagctggcgccgctctgcagatcccctttgctatgcagatggcctaccggttcaacggcatcggagtgacccagaatgtgctgtacgagaaccagaagctgatcgccaaccagttcaacagcgccatcggcaagatccaggacagcctgagcagcacagcaagcgccctgggaaagctgcaggacgtggtcaaccagaatgcccaggcactgaacaccctggtcaagcagctgtcctccaacttcggcgccatcagctctgtgctgaacgatatcctgagcagactggacaaggtggaagccgaggtgcagatcgacagactgatcaccggaaggctgcagtccctgcagacctacgttacccagcagctgatcagagccgccgagattagagcctctgccaatctggccgccaccaagatgtctgagtgtgtgctgggccagagcaagagagtggacttttgcggcaagggctaccacctgatgagcttccctcagtctgcccctcacggcgtggtgtttctgcacgtgacatacgtgcccgctcaagagaagaatttcaccaccgctccagccatctgccacgacggcaaagcccactttcctagagaaggcgtgttcgtgtccaacggcacccattggttcgtgacccagcggaacttctacgagccccagatcatcaccaccgacaacaccttcgtgtctggcaactgcgacgtcgtgatcggcattgtgaacaataccgtgtacgaccctctgcagcccgagctggacagcttcaaagaggaactggataagtactttaagaaccacacaagccccgacgtggacctgggcgatatcagcggaatcaatgccagcgtcgtgaacatccagaaagagatcgaccggctgaacgaggtggccaagaatctgaacgagagcctgatcgacctgcaagaactggggaagtacgagcagtacatcaagtggccctggtacatctggctgggctttatcgccggactgattgccatcgtgatggtcacaatcatgctgtgttgcatgaccagctgctgtagctgcctgaagggctgttgtagctgtggcagctgctgcaagttcgacgaggacgattctgagcccgtgctgaagggcgtgaaactgcactacacctga

SEQ ID NO: 2 - protein, 1273 aa, synthetic construct
  REGION 1..1273: note = Synthetic Construct
MFVFLVLLPLVSSQCVNLTTRTQLPPAYTNSFTRGVYYPDKVFRSSVLHSTQDLFLPFFSNVTWFHAIHVSGTNGTKRFDNPVLPFNDGVYFASTEKSNIIRGWIFGTTLDSKTQSLLIVNNATNVVIKVCEFQFCNDPFLGVYYHKNNKSWMESEFRVYSSANNCTFEYVSQPFLMDLEGKQGNFKNLREFVFKNIDGYFKIYSKHTPINLVRDLPQGFSALEPLVDLPIGINITRFQTLLALHRSYLTPGDSSSGWTAGAAAYYVGYLQPRTFLLKYNENGTITDAVDCALDPLSETKCTLKSFTVEKGIYQTSNFRVQPTESIVRFPNITNLCPFGEVFNATRFASVYAWNRKRISNCVADYSVLYNSASFSTFKCYGVSPTKLNDLCFTNVYADSFVIRGDEVRQIAPGQTGKIADYNYKLPDDFTGCVIAWNSNNLDSKVGGNYNYLYRLFRKSNLKPFERDISTEIYQAGSTPCNGVEGFNCYFPLQSYGFQPTNGVGYQPYRVVVLSFELLHAPATVCGPKKSTNLVKNKCVNFNFNGLTGTGVLTESNKKFLPFQQFGRDIADTTDAVRDPQTLEILDITPCSFGGVSVITPGTNTSNQVAVLYQDVNCTEVPVAIHADQLTPTWRVYSTGSNVFQTRAGCLIGAEHVNNSYECDIPIGAGICASYQTQTNSPRRARSVASQSIIAYTMSLGAENSVAYSNNSIAIPTNFTISVTTEILPVSMTKTSVDCTMYICGDSTECSNLLLQYGSFCTQLNRALTGIAVEQDKNTQEVFAQVKQIYKTPPIKDFGGFNFSQILPDPSKPSKRSFIEDLLFNKVTLADAGFIKQYGDCLGDIAARDLICAQKFNGLTVLPPLLTDEMIAQYTSALLAGTITSGWTFGAGAALQIPFAMQMAYRFNGIGVTQNVLYENQKLIANQFNSAIGKIQDSLSSTASALGKLQDVVNQNAQALNTLVKQLSSNFGAISSVLNDILSRLDKVEAEVQIDRLITGRLQSLQTYVTQQLIRAAEIRASANLAATKMSECVLGQSKRVDFCGKGYHLMSFPQSAPHGVVFLHVTYVPAQEKNFTTAPAICHDGKAHFPREGVFVSNGTHWFVTQRNFYEPQIITTDNTFVSGNCDVVIGIVNNTVYDPLQPELDSFKEELDKYFKNHTSPDVDLGDISGINASVVNIQKEIDRLNEVAKNLNESLIDLQELGKYEQYIKWPWYIWLGFIAGLIAIVMVTIMLCCMTSCCSCLKGCCSCGSCCKFDEDDSEPVLKGVKLHYT

SEQ ID NO: 3 - DNA, 585 bp, synthetic construct
  misc_feature 1..585: note = synthetic polynucleotide for RBD
  source 1..585: mol_type = other DNA
  CDS 1..585
aatatcaccaatctgtgccccttcggcgaggtgttcaatgccaccagattcgcctctgtgtacgcctggaaccggaagcggatcagcaattgcgtggccgactactccgtgctgtacaactccgccagcttcagcaccttcaagtgctacggcgtgtcccctaccaagctgaacgacctgtgcttcacaaacgtgtacgccgacagcttcgtgatccggggagatgaagtgcggcagattgcccctggacagacaggcaagatcgccgactacaactacaagctgcccgacgacttcaccggctgtgtgattgcctggaacagcaacaacctggactccaaagtcggcggcaactacaattacctgtaccggctgttccggaagtccaatctgaagcccttcgagcgggacatctccaccgagatctatcaggccggcagcaccccttgtaacggcgtggaaggcttcaactgctacttcccactgcagtcctacggctttcagcccacaaatggcgtgggctatcagccctacagagtggtggtgctgagcttcgaactgctgcatgcccctgccacagtgtga

SEQ ID NO: 4 - protein, 194 aa, synthetic construct
  REGION 1..194: note = Synthetic Construct
NITNLCPFGEVFNATRFASVYAWNRKRISNCVADYSVLYNSASFSTFKCYGVSPTKLNDLCFTNVYADSFVIRGDEVRQIAPGQTGKIADYNYKLPDDFTGCVIAWNSNNLDSKVGGNYNYLYRLFRKSNLKPFERDISTEIYQAGSTPCNGVEGFNCYFPLQSYGFQPTNGVGYQPYRVVVLSFELLHAPATV

SEQ ID NO: 5 - protein, 18 aa, synthetic construct
  REGION 1..18: note = synthetic peptide (2019-nCoV signal peptide)
MFVFLVLLPLVSSQCVNL

SEQ ID NO: 6 - protein, 26 aa, synthetic construct
  REGION 1..26: note = synthetic peptide (CD5 signal peptide)
MPMGSLQPLATLYLLGMLVASCLGRL

SEQ ID NO: 7 - protein, 19 aa, synthetic construct
  REGION 1..19: note = synthetic peptide (IL2 signal peptide)
MYRMQLLSCIALSLALVTN

SEQ ID NO: 8 - protein, 13 aa, synthetic construct
  REGION 1..13: note = synthetic peptide (PADRE epitope)
AKFVAAWTLKAAA

SEQ ID NO: 9 - protein, 4 aa, synthetic construct
  REGION 1..4: note = synthetic peptide (linker)
SGSG

SEQ ID NO: 10 - DNA, 3828 bp, synthetic construct
  misc_feature 1..3828: note = synthetic polynucleotide for Antigen_1_nCov_Spike_full_opt_h.sapiens_koz
  source 1..3828: mol_type = other DNA
  CDS 7..3828
gccaccatgttcgtgtttctggtgctgctgcctctggtgtccagccagtgtgtgaacctgaccaccagaacacagctgcctccagcctacaccaacagctttaccagaggcgtgtactaccccgacaaggtgttcagatccagcgtgctgcactctacccaggacctgttcctgcctttcttcagcaacgtgacctggttccacgccatccacgtgtccggcaccaatggcaccaagagattcgacaaccccgtgctgcccttcaacgacggggtgtactttgccagcaccgagaagtccaacatcatcagaggctggatcttcggcaccacactggacagcaagacccagagcctgctgatcgtgaacaacgccaccaacgtggtcatcaaagtgtgcgagttccagttctgcaacgaccccttcctgggcgtctactaccacaagaacaacaagagctggatggaaagcgagttccgggtgtacagcagcgccaacaactgcaccttcgagtacgtgtcccagcctttcctgatggacctggaaggcaagcagggcaacttcaagaacctgcgcgagttcgtgttcaagaacatcgacggctacttcaagatctacagcaagcacacccctatcaacctcgtgcgggatctgcctcagggcttctctgctctggaacccctggtggatctgcccatcggcatcaacatcacccggtttcagacactgctggccctgcacagaagctacctgacacctggcgatagcagcagcggatggacagctggtgccgccgcttactatgtgggctacctgcagcctagaaccttcctgctgaagtacaacgagaacggcaccatcaccgacgccgtggattgtgctctggatcctctgagcgagacaaagtgcaccctgaagtccttcaccgtggaaaagggcatctaccagaccagcaacttccgggtgcagcccaccgaatccatcgtgcggttccccaatatcaccaatctgtgccccttcggcgaggtgttcaatgccaccagattcgcctctgtgtacgcctggaaccggaagcggatcagcaattgcgtggccgactactccgtgctgtacaactccgccagcttcagcaccttcaagtgctacggcgtgtcccctaccaagctgaacgacctgtgcttcacaaacgtgtacgccgacagcttcgtgatccggggagatgaagtgcggcagattgcccctggacagacaggcaagatcgccgactacaactacaagctgcccgacgacttcaccggctgtgtgattgcctggaacagcaacaacctggactccaaagtcggcggcaactacaattacctgtaccggctgttccggaagtccaatctgaagcccttcgagcgggacatctccaccgagatctatcaggccggcagcaccccttgtaacggcgtggaaggcttcaactgctacttcccactgcagtcctacggctttcagcccacaaatggcgtgggctatcagccctacagagtggtggtgctgagcttcgaactgctgcatgcccctgccacagtgtgcggccctaagaaaagcaccaatctcgtgaagaacaaatgcgtgaacttcaacttcaacggcctgaccggcaccggcgtgctgacagagagcaacaagaagttcctgccattccagcagtttggccgggatatcgccgataccacagacgccgttagagatccccagacactggaaatcctggacatcaccccttgcagcttcggcggagtgtctgtgatcacccctggcaccaacaccagcaatcaggtggcagtgctgtaccaggacgtgaactgtaccgaagtgcccgtggccattcacgccgatcagctgacacctacatggcgggtgtactccaccggcagcaatgtgtttcagaccagagccggctgtctgatcggagccgagcacgtgaacaatagctacgagtgcgacatccccatcggcgctggcatctgtgccagctaccagacacagacaaacagccccagacgggccagatctgtggccagccagagcatcattgcctacacaatgtctctgggcgccgagaacagcgtggcctactccaacaactctatcgctatccccaccaacttcaccatcagcgtgaccacagagatcctgcctgtgtccatgaccaagaccagcgtggactgcaccatgtacatctgcggcgattccaccgagtgctccaacctgctgctgcagtacggcagcttctgcacccagctgaatagagccctgacagggatcgccgtggaacaggacaagaacacccaagaggtgttcgcccaagtgaagcagatctacaagacccctcctatcaaggacttcggcggcttcaatttcagccagattctgcccgatcctagcaagcccagcaagcggagcttcatcgaggacctgctgttcaacaaagtgacactggccgacgccggcttcatcaagcagtatggcgattgtctgggcgacattgccgccagggatctgatttgcgcccagaagtttaacggactgacagtgctgcctcctctgctgaccgatgagatgatcgcccagtacacatctgccctgctggccggcacaatcacaagcggctggacatttggagctggcgccgctctgcagatcccctttgctatgcagatggcctaccggttcaacggcatcggagtgacccagaatgtgctgtacgagaaccagaagctgatcgccaaccagttcaacagcgccatcggcaagatccaggacagcctgagcagcacagcaagcgccctgggaaagctgcaggacgtggtcaaccagaatgcccaggcactgaacaccctggtcaagcagctgtcctccaacttcggcgccatcagctctgtgctgaacgatatcctgagcagactggacaaggtggaagccgaggtgcagatcgacagactgatcaccggaaggctgcagtccctgcagacctacgttacccagcagctgatcagagccgccgagattagagcctctgccaatctggccgccaccaagatgtctgagtgtgtgctgggccagagcaagagagtggacttttgcggcaagggctaccacctgatgagcttccctcagtctgcccctcacggcgtggtgtttctgcacgtgacatacgtgcccgctcaagagaagaatttcaccaccgctccagccatctgccacgacggcaaagcccactttcctagagaaggcgtgttcgtgtccaacggcacccattggttcgtgacccagcggaacttctacgagccccagatcatcaccaccgacaacaccttcgtgtctggcaactgcgacgtcgtgatcggcattgtgaacaataccgtgtacgaccctctgcagcccgagctggacagcttcaaagaggaactggataagtactttaagaaccacacaagccccgacgtggacctgggcgatatcagcggaatcaatgccagcgtcgtgaacatccagaaagagatcgaccggctgaacgaggtggccaagaatctgaacgagagcctgatcgacctgcaagaactggggaagtacgagcagtacatcaagtggccctggtacatctggctgggctttatcgccggactgattgccatcgtgatggtcacaatcatgctgtgttgcatgaccagctgctgtagctgcctgaagggctgttgtagctgtggcagctgctgcaagttcgacgaggacgattctgagcccgtgctgaagggcgtgaaactgcactacacctga

SEQ ID NO: 11 - protein, 1273 aa, synthetic construct; identical to SEQ ID NO: 2
  REGION 1..1273: note = Synthetic Construct

SEQ ID NO: 12 - DNA, 3882 bp, synthetic construct
  misc_feature 1..3882: note = synthetic polynucleotide for Antigen_1_nCov_Spike_full_opt_h.sapiens_koz_with_nonnatural pan DR epitope (PADRE)
  source 1..3882: mol_type = other DNA
  CDS 7..3882
gccaccatgttcgtgtttctggtgctgctgcctctggtgtccagccagtgtgtgaacctgaccaccagaacacagctgcctccagcctacaccaacagctttaccagaggcgtgtactaccccgacaaggtgttcagatccagcgtgctgcactctacccaggacctgttcctgcctttcttcagcaacgtgacctggttccacgccatccacgtgtccggcaccaatggcaccaagagattcgacaaccccgtgctgcccttcaacgacggggtgtactttgccagcaccgagaagtccaacatcatcagaggctggatcttcggcaccacactggacagcaagacccagagcctgctgatcgtgaacaacgccaccaacgtggtcatcaaagtgtgcgagttccagttctgcaacgaccccttcctgggcgtctactaccacaagaacaacaagagctggatggaaagcgagttccgggtgtacagcagcgccaacaactgcaccttcgagtacgtgtcccagcctttcctgatggacctggaaggcaagcagggcaacttcaagaacctgcgcgagttcgtgttcaagaacatcgacggctacttcaagatctacagcaagcacacccctatcaacctcgtgcgggatctgcctcagggcttctctgctctggaacccctggtggatctgcccatcggcatcaacatcacccggtttcagacactgctggccctgcacagaagctacctgacacctggcgatagcagcagcggatggacagctggtgccgccgcttactatgtgggctacctgcagcctagaaccttcctgctgaagtacaacgagaacggcaccatcaccgacgccgtggattgtgctctggatcctctgagcgagacaaagtgcaccctgaagtccttcaccgtggaaaagggcatctaccagaccagcaacttccgggtgcagcccaccgaatccatcgtgcggttccccaatatcaccaatctgtgccccttcggcgaggtgttcaatgccaccagattcgcctctgtgtacgcctggaaccggaagcggatcagcaattgcgtggccgactactccgtgctgtacaactccgccagcttcagcaccttcaagtgctacggcgtgtcccctaccaagctgaacgacctgtgcttcacaaacgtgtacgccgacagcttcgtgatccggggagatgaagtgcggcagattgcccctggacagacaggcaagatcgccgactacaactacaagctgcccgacgacttcaccggctgtgtgattgcctggaacagcaacaacctggactccaaagtcggcggcaactacaattacctgtaccggctgttccggaagtccaatctgaagcccttcgagcgggacatctccaccgagatctatcaggccggcagcaccccttgtaacggcgtggaaggcttcaactgctacttcccactgcagtcctacggctttcagcccacaaatggcgtgggctatcagccctacagagtggtggtgctgagcttcgaactgctgcatgcccctgccacagtgtgcggccctaagaaaagcaccaatctcgtgaagaacaaatgcgtgaacttcaacttcaacggcctgaccggcaccggcgtgctgacagagagcaacaagaagttcctgccattccagcagtttggccgggatatcgccgataccacagacgccgttagagatccccagacactggaaatcctggacatcaccccttgcagcttcggcggagtgtctgtgatcacccctggcaccaacaccagcaatcaggtggcagtgctgtaccaggacgtgaactgtaccgaagtgcccgtggccattcacgccgatcagctgacacctacatggcgggtgtactccaccggcagcaatgtgtttcagaccagagccggctgtctgatcggagccgagcacgtgaacaatagctacgagtgcgacatccccatcggcgctggcatctgtgccagctaccagacacagacaaacagccccagacgggccagatctgtggccagccagagcatcattgcctacacaatgtctctgggcgccgagaacagcgtggcctactccaacaactctatcgctatccccaccaacttcaccatcagcgtgaccacagagatcctgcctgtgtccatgaccaagaccagcgtggactgcaccatgtacatctgcggcgattccaccgagtgctccaacctgctgctgcagtacggcagcttctgcacccagctgaatagagccctgacagggatcgccgtggaacaggacaagaacacccaagaggtgttcgcccaagtgaagcagatctacaagacccctcctatcaaggacttcggcggcttcaatttcagccagattctgcccgatcctagcaagcccagcaagcggagcttcatcgaggacctgctgttcaacaaagtgacactggccgacgccggcttcatcaagcagtatggcgattgtctgggcgacattgccgccagggatctgatttgcgcccagaagtttaacggactgacagtgctgcctcctctgctgaccgatgagatgatcgcccagtacacatctgccctgctggccggcacaatcacaagcggctggacatttggagctggcgccgctctgcagatcccctttgctatgcagatggcctaccggttcaacggcatcggagtgacccagaatgtgctgtacgagaaccagaagctgatcgccaaccagttcaacagcgccatcggcaagatccaggacagcctgagcagcacagcaagcgccctgggaaagctgcaggacgtggtcaaccagaatgcccaggcactgaacaccctggtcaagcagctgtcctccaacttcggcgccatcagctctgtgctgaacgatatcctgagcagactggacaaggtggaagccgaggtgcagatcgacagactgatcaccggaaggctgcagtccctgcagacctacgttacccagcagctgatcagagccgccgagattagagcctctgccaatctggccgccaccaagatgtctgagtgtgtgctgggccagagcaagagagtggacttttgcggcaagggctaccacctgatgagcttccctcagtctgcccctcacggcgtggtgtttctgcacgtgacatacgtgcccgctcaagagaagaatttcaccaccgctccagccatctgccacgacggcaaagcccactttcctagagaaggcgtgttcgtgtccaacggcacccattggttcgtgacccagcggaacttctacgagccccagatcatcaccaccgacaacaccttcgtgtctggcaactgcgacgtcgtgatcggcattgtgaacaataccgtgtacgaccctctgcagcccgagctggacagcttcaaagaggaactggataagtactttaagaaccacacaagccccgacgtggacctgggcgatatcagcggaatcaatgccagcgtcgtgaacatccagaaagagatcgaccggctgaacgaggtggccaagaatctgaacgagagcctgatcgacctgcaagaactggggaagtacgagcagtacatcaagtggccctggtacatctggctgggctttatcgccggactgattgccatcgtgatggtcacaatcatgctgtgttgcatgaccagctgctgtagctgcctgaagggctgttgtagctgtggcagctgctgcaagttcgacgaggacgattctgagcccgtgctgaagggcgtgaaactgcactacacctctggaagcggcgccaagtttgtggctgcctggacactgaaagccgccgcttgatga

SEQ ID NO: 13 - protein, 1290 aa, synthetic construct
  REGION 1..1290: note = Synthetic Construct
MFVFLVLLPLVSSQCVNLTTRTQLPPAYTNSFTRGVYYPDKVFRSSVLHSTQDLFLPFFSNVTWFHAIHVSGTNGTKRFDNPVLPFNDGVYFASTEKSNIIRGWIFGTTLDSKTQSLLIVNNATNVVIKVCEFQFCNDPFLGVYYHKNNKSWMESEFRVYSSANNCTFEYVSQPFLMDLEGKQGNFKNLREFVFKNIDGYFKIYSKHTPINLVRDLPQGFSALEPLVDLPIGINITRFQTLLALHRSYLTPGDSSSGWTAGAAAYYVGYLQPRTFLLKYNENGTITDAVDCALDPLSETKCTLKSFTVEKGIYQTSNFRVQPTESIVRFPNITNLCPFGEVFNATRFASVYAWNRKRISNCVADYSVLYNSASFSTFKCYGVSPTKLNDLCFTNVYADSFVIRGDEVRQIAPGQTGKIADYNYKLPDDFTGCVIAWNSNNLDSKVGGNYNYLYRLFRKSNLKPFERDISTEIYQAGSTPCNGVEGFNCYFPLQSYGFQPTNGVGYQPYRVVVLSFELLHAPATVCGPKKSTNLVKNKCVNFNFNGLTGTGVLTESNKKFLPFQQFGRDIADTTDAVRDPQTLEILDITPCSFGGVSVITPGTNTSNQVAVLYQDVNCTEVPVAIHADQLTPTWRVYSTGSNVFQTRAGCLIGAEHVNNSYECDIPIGAGICASYQTQTNSPRRARSVASQSIIAYTMSLGAENSVAYSNNSIAIPTNFTISVTTEILPVSMTKTSVDCTMYICGDSTECSNLLLQYGSFCTQLNRALTGIAVEQDKNTQEVFAQVKQIYKTPPIKDFGGFNFSQILPDPSKPSKRSFIEDLLFNKVTLADAGFIKQYGDCLGDIAARDLICAQKFNGLTVLPPLLTDEMIAQYTSALLAGTITSGWTFGAGAALQIPFAMQMAYRFNGIGVTQNVLYENQKLIANQFNSAIGKIQDSLSSTASALGKLQDVVNQNAQALNTLVKQLSSNFGAISSVLNDILSRLDKVEAEVQIDRLITGRLQSLQTYVTQQLIRAAEIRASANLAATKMSECVLGQSKRVDFCGKGYHLMSFPQSAPHGVVFLHVTYVPAQEKNFTTAPAICHDGKAHFPREGVFVSNGTHWFVTQRNFYEPQIITTDNTFVSGNCDVVIGIVNNTVYDPLQPELDSFKEELDKYFKNHTSPDVDLGDISGINASVVNIQKEIDRLNEVAKNLNESLIDLQELGKYEQYIKWPWYIWLGFIAGLIAIVMVTIMLCCMTSCCSCLKGCCSCGSCCKFDEDDSEPVLKGVKLHYTSGSGAKFVAAWTLKAAA

SEQ ID NO: 14 - DNA, 651 bp, synthetic construct
  misc_feature 1..651: note = synthetic polynucleotide for Antigen_2a_nCovRDB_SPnCov_OPT_koz
  source 1..651: mol_type = other DNA
  CDS 7..651
gccaccatgttcgtgtttctggtgctgctgcctctggtgtccagccagtgtgtgaacctggtcgctaatatcaccaatctgtgccccttcggcgaggtgttcaatgccaccagattcgcctctgtgtacgcctggaaccggaagcggatcagcaattgcgtggccgactactccgtgctgtacaactccgccagcttcagcaccttcaagtgctacggcgtgtcccctaccaagctgaacgacctgtgcttcacaaacgtgtacgccgacagcttcgtgatccggggagatgaagtgcggcagattgcccctggacagacaggcaagatcgccgactacaactacaagctgcccgacgacttcaccggctgtgtgattgcctggaacagcaacaacctggactccaaagtcggcggcaactacaattacctgtaccggctgttccggaagtccaatctgaagcccttcgagcgggacatctccaccgagatctatcaggccggcagcaccccttgtaacggcgtggaaggcttcaactgctacttcccactgcagtcctacggctttcagcccacaaatggcgtgggctatcagccctacagagtggtggtgctgagcttcgaactgctgcatgcccctgccacagtgtga

SEQ ID NO: 15 - protein, 214 aa, synthetic construct
  REGION 1..214: note = Synthetic Construct
MFVFLVLLPLVSSQCVNLVANITNLCPFGEVFNATRFASVYAWNRKRISNCVADYSVLYNSASFSTFKCYGVSPTKLNDLCFTNVYADSFVIRGDEVRQIAPGQTGKIADYNYKLPDDFTGCVIAWNSNNLDSKVGGNYNYLYRLFRKSNLKPFERDISTEIYQAGSTPCNGVEGFNCYFPLQSYGFQPTNGVGYQPYRVVVLSFELLHAPATV

SEQ ID NO: 16 - DNA, 705 bp, synthetic construct
  misc_feature 1..705: note = synthetic polynucleotide for Antigen_2a_nCovRDB_SPnCov_OPT_koz_withPADRE
  source 1..705: mol_type = other DNA
  CDS 7..705
gccaccatgttcgtgtttctggtgctgctgcctctggtgtccagccagtgtgtgaacctggtcgctaatatcaccaatctgtgccccttcggcgaggtgttcaatgccaccagattcgcctctgtgtacgcctggaaccggaagcggatcagcaattgcgtggccgactactccgtgctgtacaactccgccagcttcagcaccttcaagtgctacggcgtgtcccctaccaagctgaacgacctgtgcttcacaaacgtgtacgccgacagcttcgtgatccggggagatgaagtgcggcagattgcccctggacagacaggcaagatcgccgactacaactacaagctgcccgacgacttcaccggctgtgtgattgcctggaacagcaacaacctggactccaaagtcggcggcaactacaattacctgtaccggctgttccggaagtccaatctgaagcccttcgagcgggacatctccaccgagatctatcaggccggcagcaccccttgtaacggcgtggaaggcttcaactgctacttcccactgcagtcctacggctttcagcccacaaatggcgtgggctatcagccctacagagtggtggtgctgagcttcgaactgctgcatgcccctgccacagtgtctggaagcggcgccaagtttgtggctgcctggacactgaaagccgccgcttgatga

SEQ ID NO: 17 - protein, 231 aa, synthetic construct
  REGION 1..231: note = Synthetic Construct
MFVFLVLLPLVSSQCVNLVANITNLCPFGEVFNATRFASVYAWNRKRISNCVADYSVLYNSASFSTFKCYGVSPTKLNDLCFTNVYADSFVIRGDEVRQIAPGQTGKIADYNYKLPDDFTGCVIAWNSNNLDSKVGGNYNYLYRLFRKSNLKPFERDISTEIYQAGSTPCNGVEGFNCYFPLQSYGFQPTNGVGYQPYRVVVLSFELLHAPATVSGSGAKFVAAWTLKAAA

SEQ ID NO: 18 - DNA, 675 bp, synthetic construct
  misc_feature 1..675: note = synthetic polynucleotide for Antigen_2b_nCovRDB_SP-CD5_OPT_koz
  source 1..675: mol_type = other DNA
  CDS 7..675
gccaccatgcccatggggtctctgcaaccgctggccaccttgtacctgctggggatgctggtcgcttcctgcctcggacggctggtcgctaatatcaccaatctgtgccccttcggcgaggtgttcaatgccaccagattcgcctctgtgtacgcctggaaccggaagcggatcagcaattgcgtggccgactactccgtgctgtacaactccgccagcttcagcaccttcaagtgctacggcgtgtcccctaccaagctgaacgacctgtgcttcacaaacgtgtacgccgacagcttcgtgatccggggagatgaagtgcggcagattgcccctggacagacaggcaagatcgccgactacaactacaagctgcccgacgacttcaccggctgtgtgattgcctggaacagcaacaacctggactccaaagtcggcggcaactacaattacctgtaccggctgttccggaagtccaatctgaagcccttcgagcgggacatctccaccgagatctatcaggccggcagcaccccttgtaacggcgtggaaggcttcaactgctacttcccactgcagtcctacggctttcagcccacaaatggcgtgggctatcagccctacagagtggtggtgctgagcttcgaactgctgcatgcccctgccacagtgtga

SEQ ID NO: 19 - protein, 222 aa, synthetic construct
  REGION 1..222: note = Synthetic Construct
MPMGSLQPLATLYLLGMLVASCLGRLVANITNLCPFGEVFNATRFASVYAWNRKRISNCVADYSVLYNSASFSTFKCYGVSPTKLNDLCFTNVYADSFVIRGDEVRQIAPGQTGKIADYNYKLPDDFTGCVIAWNSNNLDSKVGGNYNYLYRLFRKSNLKPFERDISTEIYQAGSTPCNGVEGFNCYFPLQSYGFQPTNGVGYQPYRVVVLSFELLHAPATV

SEQ ID NO: 20 - DNA, 729 bp, synthetic construct
  misc_feature 1..729: note = synthetic polynucleotide for Antigen_2b_nCovRDB_SP-CD5_OPT_koz_withPADRE
  source 1..729: mol_type = other DNA
  CDS 7..729
gccaccatgcccatggggtctctgcaaccgctggccaccttgtacctgctggggatgctggtcgcttcctgcctcggacggctggtcgctaatatcaccaatctgtgccccttcggcgaggtgttcaatgccaccagattcgcctctgtgtacgcctggaaccggaagcggatcagcaattgcgtggccgactactccgtgctgtacaactccgccagcttcagcaccttcaagtgctacggcgtgtcccctaccaagctgaacgacctgtgcttcacaaacgtgtacgccgacagcttcgtgatccggggagatgaagtgcggcagattgcccctggacagacaggcaagatcgccgactacaactacaagctgcccgacgacttcaccggctgtgtgattgcctggaacagcaacaacctggactccaaagtcggcggcaactacaattacctgtaccggctgttccggaagtccaatctgaagcccttcgagcgggacatctccaccgagatctatcaggccggcagcaccccttgtaacggcgtggaaggcttcaactgctacttcccactgcagtcctacggctttcagcccacaaatggcgtgggctatcagccctacagagtggtggtgctgagcttcgaactgctgcatgcccctgccacagtgtctggaagcggcgccaagtttgtggctgcctggacactgaaagccgccgcttgatga

SEQ ID NO: 21 - protein, 239 aa, synthetic construct
  REGION 1..239: note = Synthetic Construct
MPMGSLQPLATLYLLGMLVASCLGRLVANITNLCPFGEVFNATRFASVYAWNRKRISNCVADYSVLYNSASFSTFKCYGVSPTKLNDLCFTNVYADSFVIRGDEVRQIAPGQTGKIADYNYKLPDDFTGCVIAWNSNNLDSKVGGNYNYLYRLFRKSNLKPFERDISTEIYQAGSTPCNGVEGFNCYFPLQSYGFQPTNGVGYQPYRVVVLSFELLHAPATVSGSGAKFVAAWTLKAAA

SEQ ID NO: 22 - DNA, 654 bp, synthetic construct
  misc_feature 1..654: note = synthetic polynucleotide for Antigen_2c_nCovRDB_SP-IL2_OPT_koz
  source 1..654: mol_type = other DNA
  CDS 7..654
gccaccatgtacaggatgcaactcctgtcttgcattgcactaagtcttgcacttgtcacaaacagtgcaaatatcaccaatctgtgccccttcggcgaggtgttcaatgccaccagattcgcctctgtgtacgcctggaaccggaagcggatcagcaattgcgtggccgactactccgtgctgtacaactccgccagcttcagcaccttcaagtgctacggcgtgtcccctaccaagctgaacgacctgtgcttcacaaacgtgtacgccgacagcttcgtgatccggggagatgaagtgcggcagattgcccctggacagacaggcaagatcgccgactacaactacaagctgcccgacgacttcaccggctgtgtgattgcctggaacagcaacaacctggactccaaagtcggcggcaactacaattacctgtaccggctgttccggaagtccaatctgaagcccttcgagcgggacatctccaccgagatctatcaggccggcagcaccccttgtaacggcgtggaaggcttcaactgctacttcccactgcagtcctacggctttcagcccacaaatggcgtgggctatcagccctacagagtggtggtgctgagcttcgaactgctgcatgcccctgccacagtgtga

SEQ ID NO: 23 - protein, 215 aa, synthetic construct
  REGION 1..215: note = Synthetic Construct
MYRMQLLSCIALSLALVTNSANITNLCPFGEVFNATRFASVYAWNRKRISNCVADYSVLYNSASFSTFKCYGVSPTKLNDLCFTNVYADSFVIRGDEVRQIAPGQTGKIADYNYKLPDDFTGCVIAWNSNNLDSKVGGNYNYLYRLFRKSNLKPFERDISTEIYQAGSTPCNGVEGFNCYFPLQSYGFQPTNGVGYQPYRVVVLSFELLHAPATV

SEQ ID NO: 24 - DNA, 708 bp, synthetic construct
  misc_feature 1..708: note = synthetic polynucleotide for Antigen_2c_nCovRDB_SP-IL2_OPT_kozwithPADRE
  source 1..708: mol_type = other DNA
  CDS 7..708
gccaccatgtacaggatgcaactcctgtcttgcattgcactaagtcttgcacttgtcacaaacagtgcaaatatcaccaatctgtgccccttcggcgaggtgttcaatgccaccagattcgcctctgtgtacgcctggaaccggaagcggatcagcaattgcgtggccgactactccgtgctgtacaactccgccagcttcagcaccttcaagtgctacggcgtgtcccctaccaagctgaacgacctgtgcttcacaaacgtgtacgccgacagcttcgtgatccggggagatgaagtgcggcagattgcccctggacagacaggcaagatcgccgactacaactacaagctgcccgacgacttcaccggctgtgtgattgcctggaacagcaacaacctggactccaaagtcggcggcaactacaattacctgtaccggctgttccggaagtccaatctgaagcccttcgagcgggacatctccaccgagatctatcaggccggcagcaccccttgtaacggcgtggaaggcttcaactgctacttcccactgcagtcctacggctttcagcccacaaatggcgtgggctatcagccctacagagtggtggtgctgagcttcgaactgctgcatgcccctgccacagtgtctggaagcggcgccaagtttgtggctgcctggacactgaaagccgccgcttgatga

SEQ ID NO: 25 - protein, 232 aa, synthetic construct
  REGION 1..232: note = Synthetic Construct
MYRMQLLSCIALSLALVTNSANITNLCPFGEVFNATRFASVYAWNRKRISNCVADYSVLYNSASFSTFKCYGVSPTKLNDLCFTNVYADSFVIRGDEVRQIAPGQTGKIADYNYKLPDDFTGCVIAWNSNNLDSKVGGNYNYLYRLFRKSNLKPFERDISTEIYQAGSTPCNGVEGFNCYFPLQSYGFQPTNGVGYQPYRVVVLSFELLHAPATVSGSGAKFVAAWTLKAAA

SEQ ID NO: 26 - DNA, 51 bp, synthetic construct
  misc_feature 1..51: note = ynthetic polynucleotide for padre_seq_OPT_nt
  source 1..51: mol_type = other DNA
  CDS 1..51
tctggaagcggcgccaagtttgtggctgcctggacactgaaagccgccgct

SEQ ID NO: 27 - protein, 17 aa, synthetic construct
  REGION 1..17: note = Synthetic Construct
SGSGAKFVAAWTLKAAA

SEQ ID NO: 28 - protein, 1196 aa, synthetic construct
  REGION 1..1196: note = synthetic polypeptide (6acd.1.A)
MFIFLLFLTLTSGSDLDRCTTFDDVQAPNYTQHTSSMRGVYYPDEIFRSDTLYLTQDLFLPFYSNVTGFHTINHTFGNPVIPFKDGIYFAATEKSNVVRGWVFGSTMNNKSQSVIIINNSTNVVIRACNFELCDNPFFAVSKPMGTQTHTMIFDNAFNCTFEYISDAFSLDVSEKSGNFKHLREFVFKNKDGFLYVYKGYQPIDVVRDLPSGFNTLKPIFKLPLGINITNFRAILTAFSPAQDIWGTSAAAYFVGYLKPTTFMLKYDENGTITDAVDCSQNPLAELKCSVKSFEIDKGIYQTSNFRVVPSGDVVRFPNITNLCPFGEVFNATKFPSVYAWERKKISNCVADYSVLYNSTFFSTFKCYGVSATKLNDLCFSNVYADSFVVKGDDVRQIAPGQTGVIADYNYKLPDDFMGCVLAWNTRNIDATSTGNYNYKYRYLRHGKLRPFERDISNVPFSPDGKPCTPPALNCYWPLNDYGFYTTTGIGYQPYRVVVLSFELLNAPATVCGPKLSTDLIKNQCVNFNFNGLTGTGVLTPSSKRFQPFQQFGRDVSDFTDSVRDPKTSEILDISPCSFGGVSVITPGTNASSEVAVLYQDVNCTDVSTAIHADQLTPAWRIYSTGNNVFQTQAGCLIGAEHVDTSYECDIPIGAGICASYHTVSLLRSTSQKSIVAYTMSLGADSSIAYSNNTIAIPTNFSISITTEVMPVSMAKTSVDCNMYICGDSTECANLLLQYGSFCTQLNRALSGIAAEQDRNTREVFAQVKQMYKTPTLKYFGGFNFSQILPDPLKPTKRSFIEDLLFNKVTLADAGFMKQYGECLGDINARDLICAQKFNGLTVLPPLLTDDMIAAYTAALVSGTATAGWTFGAGAALQIPFAMQMAYRFNGIGVTQNVLYENQKQIANQFNKAISQIQESLTTTSTALGKLQDVVNQNAQALNTLVKQLSSNFGAISSVLNDILSRLDKVEAEVQIDRLITGRLQSLQTYVTQQLIRAAEIRASANLAATKMSECVLGQSKRVDFCGKGYHLMSFPQAAPHGVVFLHVTYVPSQERNFTTAPAICHEGKAYFPREGVFVFNGTSWFITQRNFFSPQIITTDNTFVSGNCDVVIGIINNTVYDPLQPELDSFKEELDKYFKNHTSPDVDLGDISGINASVVNIQKEIDRLNEVAKNLNESLIDLQELGKYEQYIKWPW

SEQ ID NO: 29 - DNA, 3828 bp, synthetic construct
  misc_feature 1..3828: note = synthetic polynucleotide encoding antigen_XXX_nCov_Spike_full_opt_h.sapiens_koz_deltaFurin
  source 1..3828: mol_type = other DNA
  CDS 7..3828
gccaccatgttcgtgtttctggtgctgctgcctctggtgtccagccagtgtgtgaacctgaccaccagaacacagctgcctccagcctacaccaacagctttaccagaggcgtgtactaccccgacaaggtgttcagatccagcgtgctgcactctacccaggacctgttcctgcctttcttcagcaacgtgacctggttccacgccatccacgtgtccggcaccaatggcaccaagagattcgacaaccccgtgctgcccttcaacgacggggtgtactttgccagcaccgagaagtccaacatcatcagaggctggatcttcggcaccacactggacagcaagacccagagcctgctgatcgtgaacaacgccaccaacgtggtcatcaaagtgtgcgagttccagttctgcaacgaccccttcctgggcgtctactaccacaagaacaacaagagctggatggaaagcgagttccgggtgtacagcagcgccaacaactgcaccttcgagtacgtgtcccagcctttcctgatggacctggaaggcaagcagggcaacttcaagaacctgcgcgagttcgtgttcaagaacatcgacggctacttcaagatctacagcaagcacacccctatcaacctcgtgcgggatctgcctcagggcttctctgctctggaacccctggtggatctgcccatcggcatcaacatcacccggtttcagacactgctggccctgcacagaagctacctgacacctggcgatagcagcagcggatggacagctggtgccgccgcttactatgtgggctacctgcagcctagaaccttcctgctgaagtacaacgagaacggcaccatcaccgacgccgtggattgtgctctggatcctctgagcgagacaaagtgcaccctgaagtccttcaccgtggaaaagggcatctaccagaccagcaacttccgggtgcagcccaccgaatccatcgtgcggttccccaatatcaccaatctgtgccccttcggcgaggtgttcaatgccaccagattcgcctctgtgtacgcctggaaccggaagcggatcagcaattgcgtggccgactactccgtgctgtacaactccgccagcttcagcaccttcaagtgctacggcgtgtcccctaccaagctgaacgacctgtgcttcacaaacgtgtacgccgacagcttcgtgatccggggagatgaagtgcggcagattgcccctggacagacaggcaagatcgccgactacaactacaagctgcccgacgacttcaccggctgtgtgattgcctggaacagcaacaacctggactccaaagtcggcggcaactacaattacctgtaccggctgttccggaagtccaatctgaagcccttcgagcgggacatctccaccgagatctatcaggccggcagcaccccttgtaacggcgtggaaggcttcaactgctacttcccactgcagtcctacggctttcagcccacaaatggcgtgggctatcagccctacagagtggtggtgctgagcttcgaactgctgcatgcccctgccacagtgtgcggccctaagaaaagcaccaatctcgtgaagaacaaatgcgtgaacttcaacttcaacggcctgaccggcaccggcgtgctgacagagagcaacaagaagttcctgccattccagcagtttggccgggatatcgccgataccacagacgccgttagagatccccagacactggaaatcctggacatcaccccttgcagcttcggcggagtgtctgtgatcacccctggcaccaacaccagcaatcaggtggcagtgctgtaccaggacgtgaactgtaccgaagtgcccgtggccattcacgccgatcagctgacacctacatggcgggtgtactccaccggcagcaatgtgtttcagaccagagccggctgtctgatcggagccgagcacgtgaacaatagctacgagtgcgacatccccatcggcgctggcatctgtgccagctaccagacacagacaaacagccccggaagcgccagctctgtggccagccagagcatcattgcctacacaatgtctctgggcgccgagaacagcgtggcctactccaacaactctatcgctatccccaccaacttcaccatcagcgtgaccacagagatcctgcctgtgtccatgaccaagaccagcgtggactgcaccatgtacatctgcggcgattccaccgagtgctccaacctgctgctgcagtacggcagcttctgcacccagctgaatagagccctgacagggatcgccgtggaacaggacaagaacacccaagaggtgttcgcccaagtgaagcagatctacaagacccctcctatcaaggacttcggcggcttcaatttcagccagattctgcccgatcctagcaagcccagcaagcggagcttcatcgaggacctgctgttcaacaaagtgacactggccgacgccggcttcatcaagcagtatggcgattgtctgggcgacattgccgccagggatctgatttgcgcccagaagtttaacggactgacagtgctgcctcctctgctgaccgatgagatgatcgcccagtacacatctgccctgctggccggcacaatcacaagcggctggacatttggagctggcgccgctctgcagatcccctttgctatgcagatggcctaccggttcaacggcatcggagtgacccagaatgtgctgtacgagaaccagaagctgatcgccaaccagttcaacagcgccatcggcaagatccaggacagcctgagcagcacagcaagcgccctgggaaagctgcaggacgtggtcaaccagaatgcccaggcactgaacaccctggtcaagcagctgtcctccaacttcggcgccatcagctctgtgctgaacgatatcctgagcagactggacaaggtggaagccgaggtgcagatcgacagactgatcaccggaaggctgcagtccctgcagacctacgttacccagcagctgatcagagccgccgagattagagcctctgccaatctggccgccaccaagatgtctgagtgtgtgctgggccagagcaagagagtggacttttgcggcaagggctaccacctgatgagcttccctcagtctgcccctcacggcgtggtgtttctgcacgtgacatacgtgcccgctcaagagaagaatttcaccaccgctccagccatctgccacgacggcaaagcccactttcctagagaaggcgtgttcgtgtccaacggcacccattggttcgtgacccagcggaacttctacgagccccagatcatcaccaccgacaacaccttcgtgtctggcaactgcgacgtcgtgatcggcattgtgaacaataccgtgtacgaccctctgcagcccgagctggacagcttcaaagaggaactggataagtactttaagaaccacacaagccccgacgtggacctgggcgatatcagcggaatcaatgccagcgtcgtgaacatccagaaagagatcgaccggctgaacgaggtggccaagaatctgaacgagagcctgatcgacctgcaagaactggggaagtacgagcagtacatcaagtggccctggtacatctggctgggctttatcgccggactgattgccatcgtgatggtcacaatcatgctgtgttgcatgaccagctgctgtagctgcctgaagggctgttgtagctgtggcagctgctgcaagttcgacgaggacgattctgagcccgtgctgaagggcgtgaaactgcactacacctga

SEQ ID NO: 30 - protein, 1273 aa, synthetic construct
  REGION 1..1273: note = Synthetic Construct
MFVFLVLLPLVSSQCVNLTTRTQLPPAYTNSFTRGVYYPDKVFRSSVLHSTQDLFLPFFSNVTWFHAIHVSGTNGTKRFDNPVLPFNDGVYFASTEKSNIIRGWIFGTTLDSKTQSLLIVNNATNVVIKVCEFQFCNDPFLGVYYHKNNKSWMESEFRVYSSANNCTFEYVSQPFLMDLEGKQGNFKNLREFVFKNIDGYFKIYSKHTPINLVRDLPQGFSALEPLVDLPIGINITRFQTLLALHRSYLTPGDSSSGWTAGAAAYYVGYLQPRTFLLKYNENGTITDAVDCALDPLSETKCTLKSFTVEKGIYQTSNFRVQPTESIVRFPNITNLCPFGEVFNATRFASVYAWNRKRISNCVADYSVLYNSASFSTFKCYGVSPTKLNDLCFTNVYADSFVIRGDEVRQIAPGQTGKIADYNYKLPDDFTGCVIAWNSNNLDSKVGGNYNYLYRLFRKSNLKPFERDISTEIYQAGSTPCNGVEGFNCYFPLQSYGFQPTNGVGYQPYRVVVLSFELLHAPATVCGPKKSTNLVKNKCVNFNFNGLTGTGVLTESNKKFLPFQQFGRDIADTTDAVRDPQTLEILDITPCSFGGVSVITPGTNTSNQVAVLYQDVNCTEVPVAIHADQLTPTWRVYSTGSNVFQTRAGCLIGAEHVNNSYECDIPIGAGICASYQTQTNSPGSASSVASQSIIAYTMSLGAENSVAYSNNSIAIPTNFTISVTTEILPVSMTKTSVDCTMYICGDSTECSNLLLQYGSFCTQLNRALTGIAVEQDKNTQEVFAQVKQIYKTPPIKDFGGFNFSQILPDPSKPSKRSFIEDLLFNKVTLADAGFIKQYGDCLGDIAARDLICAQKFNGLTVLPPLLTDEMIAQYTSALLAGTITSGWTFGAGAALQIPFAMQMAYRFNGIGVTQNVLYENQKLIANQFNSAIGKIQDSLSSTASALGKLQDVVNQNAQALNTLVKQLSSNFGAISSVLNDILSRLDKVEAEVQIDRLITGRLQSLQTYVTQQLIRAAEIRASANLAATKMSECVLGQSKRVDFCGKGYHLMSFPQSAPHGVVFLHVTYVPAQEKNFTTAPAICHDGKAHFPREGVFVSNGTHWFVTQRNFYEPQIITTDNTFVSGNCDVVIGIVNNTVYDPLQPELDSFKEELDKYFKNHTSPDVDLGDISGINASVVNIQKEIDRLNEVAKNLNESLIDLQELGKYEQYIKWPWYIWLGFIAGLIAIVMVTIMLCCMTSCCSCLKGCCSCGSCCKFDEDDSEPVLKGVKLHYT

SEQ ID NO: 31 - DNA, 651 bp, synthetic construct
  misc_feature 1..651: note = synthetic polynucleotide encoding antigen_2a_nCovRDB_SPnCov_OPT_koz_Var1
  source 1..651: mol_type = other DNA
  CDS 7..651
gccaccatgttcgtgtttctggtgctgctgcctctggtgtccagccagtgtgtgaacctggtcgctaatatcaccaatctgtgccccttcggcgaggtgttcaatgccaccagattcgcctctgtgtacgcctggaaccggaagcggatcagcaattgcgtggccgactactccgtgctgtacaactccgccagcttcagcaccttcaagtgctacggcgtgtcccctaccaagctgaacgacctgtgcttcacaaacgtatacgccgacagcttcgtgatccggggagatgaagtgcggcagattgcccctggacagacaggcaagatcgccgactacaactacaagctgcccgacgacttcaccggctgtgtgattgcctggaacagcaacaacctggactccaaagtcggcggcaactacaattacctgtaccggctgttccggaagtccaatctgaagcccttcgagcgggacatctccaccgagatctatcaggccggcagcaccccttgtaacggcgtgaaaggcttcaactgctacttcccactgcagtcctacggctttcagcccacatatggcgtgggctatcagccctacagagtggtggtgctgagcttcgaactgctgcatgcccctgccacagtgtga

SEQ ID NO: 32 - protein, 214 aa, synthetic construct
  REGION 1..214: note = Synthetic Construct
MFVFLVLLPLVSSQCVNLVANITNLCPFGEVFNATRFASVYAWNRKRISNCVADYSVLYNSASFSTFKCYGVSPTKLNDLCFTNVYADSFVIRGDEVRQIAPGQTGKIADYNYKLPDDFTGCVIAWNSNNLDSKVGGNYNYLYRLFRKSNLKPFERDISTEIYQAGSTPCNGVKGFNCYFPLQSYGFQPTYGVGYQPYRVVVLSFELLHAPATV

SEQ ID NO: 33 - DNA, 651 bp, synthetic construct
  misc_feature 1..651: note = synthetic polynucleotide encoding antigen_2a_nCovRDB_SPnCov_OPT_koz_Var2
  source 1..651: mol_type = other DNA
  CDS 7..651
gccaccatgttcgtgtttctggtgctgctgcctctggtgtccagccagtgtgtgaacctggtcgctaatatcaccaatctgtgccccttcggcgaggtgttcaatgccaccagattcgcctctgtgtacgcctggaaccggaagcggatcagcaattgcgtggccgactactccgtgctgtacaactccgccagcttcagcaccttcaagtgctacggcgtgtcccctaccaagctgaacgacctgtgcttcacaaacgtgtacgccgacagcttcgtgatccggggagatgaagtgcggcagattgcccctggacagacaggcaatatcgccgactacaactacaagctgcccgacgacttcaccggctgtgtgattgcctggaacagcaacaacctggactccaaagtcggcggcaactacaattacctgtaccggctgttccggaagtccaatctgaagcccttcgagcgggacatctccaccgagatctatcaggccggcagcaccccttgtaacggcgtgaaaggcttcaactgctacttcccactgcagtcctacggctttcagcccacatatggcgtgggctatcagccctacagagtggtggtgctgagcttcgaactgctgcatgcccctgccacagtgtga

SEQ ID NO: 34 - protein, 214 aa, synthetic construct
  REGION 1..214: note = Synthetic Construct
MFVFLVLLPLVSSQCVNLVANITNLCPFGEVFNATRFASVYAWNRKRISNCVADYSVLYNSASFSTFKCYGVSPTKLNDLCFTNVYADSFVIRGDEVRQIAPGQTGNIADYNYKLPDDFTGCVIAWNSNNLDSKVGGNYNYLYRLFRKSNLKPFERDISTEIYQAGSTPCNGVKGFNCYFPLQSYGFQPTYGVGYQPYRVVVLSFELLHAPATV

SEQ ID NO: 35 - DNA, 651 bp, synthetic construct
  misc_feature 1..651: note = synthetic polynucleotide encoding antigen_2a_nCovRDB_SPnCov_OPT_koz_Var3
  source 1..651: mol_type = other DNA
  CDS 7..651
gccaccatgttcgtgtttctggtgctgctgcctctggtgtccagccagtgtgtgaacctggtcgctaatatcaccaatctgtgccccttcggcgaggtgttcaatgccaccagattcgcctctgtgtacgcctggaaccggaagcggatcagcaattgcgtggccgactactccgtgctgtacaactccgccagcttcagcaccttcaagtgctacggcgtgtcccctaccaagctgaacgacctgtgcttcacaaacgtatacgccgacagcttcgtgatccggggagatgaagtgcggcagattgcccctggacagacaggcaatatcgccgactacaactacaagctgcccgacgacttcaccggctgtgtgattgcctggaacagcaagaacctggactccaaagtcggcggcaactacaattacctgttccggctgttccggaagtccaatctgaagcccttcgagcgggacatctccaccgagatctatcaggccggcaacaccccttgtaacggcgtgaaaggcttcaactgctactccccactgcagtcctacggctttcagcccacatatggcgtgggctatcagccctacagagtggtggtgctgagcttcgaactgctgcatgcccctgccacagtgtga

SEQ ID NO: 36 - protein, 214 aa, synthetic construct
  REGION 1..214: note = Synthetic Construct
MFVFLVLLPLVSSQCVNLVANITNLCPFGEVFNATRFASVYAWNRKRISNCVADYSVLYNSASFSTFKCYGVSPTKLNDLCFTNVYADSFVIRGDEVRQIAPGQTGNIADYNYKLPDDFTGCVIAWNSKNLDSKVGGNYNYLFRLFRKSNLKPFERDISTEIYQAGNTPCNGVKGFNCYSPLQSYGFQPTYGVGYQPYRVVVLSFELLHAPATV

SEQ ID NO: 37 - DNA, 651 bp, synthetic construct
  misc_feature 1..651: note = synthetic polynucleotide coding for Antigen_2a_nCovRDB_SPnCov_OPT_koz_Var4
  source 1..651: mol_type = other DNA
  CDS 7..651
gccaccatgttcgtgtttctggtgctgctgcctctggtgtccagccagtgtgtgaacctggtcgctaatatcaccaatctgtgccccttcggcgaggtgttcaatgccaccagattcgcctctgtgtacgcctggaaccggaagcggatcagcaattgcgtggccgactactccgtgctgtacaactccgccagcttcagcaccttcaagtgctacggcgtgtcccctaccaagctgaacgacctgtgcttcacaaacgtatacgccgacagcttcgtgatccggggagatgaagtgcggcagattgcccctggacagacaggcaatatcgccgactacaactacaagctgcccgacgacttcaccggctgtgtgattgcctggaacagcaagaacctggactccaaagtcggcggcaactacaattaccggtaccggctgttccggaagtccaatctgaagcccttcgagcgggacatctccaccgagatctatcaggccggcaacaccccttgtaacggcgtgaaaggcttcaactgctactccccactgcagtcctacggctttcagcccacatatggcgtgggctatcagccctacagagtggtggtgctgagcttcgaactgctgcatgcccctgccacagtgtga

SEQ ID NO: 38 - protein, 214 aa, synthetic construct
  REGION 1..214: note = Synthetic Construct
MFVFLVLLPLVSSQCVNLVANITNLCPFGEVFNATRFASVYAWNRKRISNCVADYSVLYNSASFSTFKCYGVSPTKLNDLCFTNVYADSFVIRGDEVRQIAPGQTGNIADYNYKLPDDFTGCVIAWNSKNLDSKVGGNYNYRYRLFRKSNLKPFERDISTEIYQAGNTPCNGVKGFNCYSPLQSYGFQPTYGVGYQPYRVVVLSFELLHAPATV

SEQ ID NO: 39 - DNA, 3771 bp, synthetic construct
  misc_feature 1..3771: note = synthetic polynucleotide for Antigen_1_nCov_Spike_full_opt_h.sapiens_koz_delta_Cter
  source 1..3771: mol_type = other DNA
  CDS 7..3771
gccaccatgttcgtgtttctggtgctgctgcctctggtgtccagccagtgtgtgaacctgaccaccagaacacagctgcctccagcctacaccaacagctttaccagaggcgtgtactaccccgacaaggtgttcagatccagcgtgctgcactctacccaggacctgttcctgcctttcttcagcaacgtgacctggttccacgccatccacgtgtccggcaccaatggcaccaagagattcgacaaccccgtgctgcccttcaacgacggggtgtactttgccagcaccgagaagtccaacatcatcagaggctggatcttcggcaccacactggacagcaagacccagagcctgctgatcgtgaacaacgccaccaacgtggtcatcaaagtgtgcgagttccagttctgcaacgaccccttcctgggcgtctactaccacaagaacaacaagagctggatggaaagcgagttccgggtgtacagcagcgccaacaactgcaccttcgagtacgtgtcccagcctttcctgatggacctggaaggcaagcagggcaacttcaagaacctgcgcgagttcgtgttcaagaacatcgacggctacttcaagatctacagcaagcacacccctatcaacctcgtgcgggatctgcctcagggcttctctgctctggaacccctggtggatctgcccatcggcatcaacatcacccggtttcagacactgctggccctgcacagaagctacctgacacctggcgatagcagcagcggatggacagctggtgccgccgcttactatgtgggctacctgcagcctagaaccttcctgctgaagtacaacgagaacggcaccatcaccgacgccgtggattgtgctctggatcctctgagcgagacaaagtgcaccctgaagtccttcaccgtggaaaagggcatctaccagaccagcaacttccgggtgcagcccaccgaatccatcgtgcggttccccaatatcaccaatctgtgccccttcggcgaggtgttcaatgccaccagattcgcctctgtgtacgcctggaaccggaagcggatcagcaattgcgtggccgactactccgtgctgtacaactccgccagcttcagcaccttcaagtgctacggcgtgtcccctaccaagctgaacgacctgtgcttcacaaacgtgtacgccgacagcttcgtgatccggggagatgaagtgcggcagattgcccctggacagacaggcaagatcgccgactacaactacaagctgcccgacgacttcaccggctgtgtgattgcctggaacagcaacaacctggactccaaagtcggcggcaactacaattacctgtaccggctgttccggaagtccaatctgaagcccttcgagcgggacatctccaccgagatctatcaggccggcagcaccccttgtaacggcgtggaaggcttcaactgctacttcccactgcagtcctacggctttcagcccacaaatggcgtgggctatcagccctacagagtggtggtgctgagcttcgaactgctgcatgcccctgccacagtgtgcggccctaagaaaagcaccaatctcgtgaagaacaaatgcgtgaacttcaacttcaacggcctgaccggcaccggcgtgctgacagagagcaacaagaagttcctgccattccagcagtttggccgggatatcgccgataccacagacgccgttagagatccccagacactggaaatcctggacatcaccccttgcagcttcggcggagtgtctgtgatcacccctggcaccaacaccagcaatcaggtggcagtgctgtaccaggacgtgaactgtaccgaagtgcccgtggccattcacgccgatcagctgacacctacatggcgggtgtactccaccggcagcaatgtgtttcagaccagagccggctgtctgatcggagccgagcacgtgaacaatagctacgagtgcgacatccccatcggcgctggcatctgtgccagctaccagacacagacaaacagccccagacgggccagatctgtggccagccagagcatcattgcctacacaatgtctctgggcgccgagaacagcgtggcctactccaacaactctatcgctatccccaccaacttcaccatcagcgtgaccacagagatcctgcctgtgtccatgaccaagaccagcgtggactgcaccatgtacatctgcggcgattccaccgagtgctccaacctgctgctgcagtacggcagcttctgcacccagctgaatagagccctgacagggatcgccgtggaacaggacaagaacacccaagaggtgttcgcccaagtgaagcagatctacaagacccctcctatcaaggacttcggcggcttcaatttcagccagattctgcccgatcctagcaagcccagcaagcggagcttcatcgaggacctgctgttcaacaaagtgacactggccgacgccggcttcatcaagcagtatggcgattgtctgggcgacattgccgccagggatctgatttgcgcccagaagtttaacggactgacagtgctgcctcctctgctgaccgatgagatgatcgcccagtacacatctgccctgctggccggcacaatcacaagcggctggacatttggagctggcgccgctctgcagatcccctttgctatgcagatggcctaccggttcaacggcatcggagtgacccagaatgtgctgtacgagaaccagaagctgatcgccaaccagttcaacagcgccatcggcaagatccaggacagcctgagcagcacagcaagcgccctgggaaagctgcaggacgtggtcaaccagaatgcccaggcactgaacaccctggtcaagcagctgtcctccaacttcggcgccatcagctctgtgctgaacgatatcctgagcagactggacaaggtggaagccgaggtgcagatcgacagactgatcaccggaaggctgcagtccctgcagacctacgttacccagcagctgatcagagccgccgagattagagcctctgccaatctggccgccaccaagatgtctgagtgtgtgctgggccagagcaagagagtggacttttgcggcaagggctaccacctgatgagcttccctcagtctgcccctcacggcgtggtgtttctgcacgtgacatacgtgcccgctcaagagaagaatttcaccaccgctccagccatctgccacgacggcaaagcccactttcctagagaaggcgtgttcgtgtccaacggcacccattggttcgtgacccagcggaacttctacgagccccagatcatcaccaccgacaacaccttcgtgtctggcaactgcgacgtcgtgatcggcattgtgaacaataccgtgtacgaccctctgcagcccgagctggacagcttcaaagaggaactggataagtactttaagaaccacacaagccccgacgtggacctgggcgatatcagcggaatcaatgccagcgtcgtgaacatccagaaagagatcgaccggctgaacgaggtggccaagaatctgaacgagagcctgatcgacctgcaagaactggggaagtacgagcagtacatcaagtggccctggtacatctggctgggctttatcgccggactgattgccatcgtgatggtcacaatcatgctgtgttgcatgaccagctgctgtagctgcctgaagggctgttgtagctgtggcagctgctgctga

SEQ ID NO: 40 - protein, 1254 aa, synthetic construct
  REGION 1..1254: note = Synthetic Construct
MFVFLVLLPLVSSQCVNLTTRTQLPPAYTNSFTRGVYYPDKVFRSSVLHSTQDLFLPFFSNVTWFHAIHVSGTNGTKRFDNPVLPFNDGVYFASTEKSNIIRGWIFGTTLDSKTQSLLIVNNATNVVIKVCEFQFCNDPFLGVYYHKNNKSWMESEFRVYSSANNCTFEYVSQPFLMDLEGKQGNFKNLREFVFKNIDGYFKIYSKHTPINLVRDLPQGFSALEPLVDLPIGINITRFQTLLALHRSYLTPGDSSSGWTAGAAAYYVGYLQPRTFLLKYNENGTITDAVDCALDPLSETKCTLKSFTVEKGIYQTSNFRVQPTESIVRFPNITNLCPFGEVFNATRFASVYAWNRKRISNCVADYSVLYNSASFSTFKCYGVSPTKLNDLCFTNVYADSFVIRGDEVRQIAPGQTGKIADYNYKLPDDFTGCVIAWNSNNLDSKVGGNYNYLYRLFRKSNLKPFERDISTEIYQAGSTPCNGVEGFNCYFPLQSYGFQPTNGVGYQPYRVVVLSFELLHAPATVCGPKKSTNLVKNKCVNFNFNGLTGTGVLTESNKKFLPFQQFGRDIADTTDAVRDPQTLEILDITPCSFGGVSVITPGTNTSNQVAVLYQDVNCTEVPVAIHADQLTPTWRVYSTGSNVFQTRAGCLIGAEHVNNSYECDIPIGAGICASYQTQTNSPRRARSVASQSIIAYTMSLGAENSVAYSNNSIAIPTNFTISVTTEILPVSMTKTSVDCTMYICGDSTECSNLLLQYGSFCTQLNRALTGIAVEQDKNTQEVFAQVKQIYKTPPIKDFGGFNFSQILPDPSKPSKRSFIEDLLFNKVTLADAGFIKQYGDCLGDIAARDLICAQKFNGLTVLPPLLTDEMIAQYTSALLAGTITSGWTFGAGAALQIPFAMQMAYRFNGIGVTQNVLYENQKLIANQFNSAIGKIQDSLSSTASALGKLQDVVNQNAQALNTLVKQLSSNFGAISSVLNDILSRLDKVEAEVQIDRLITGRLQSLQTYVTQQLIRAAEIRASANLAATKMSECVLGQSKRVDFCGKGYHLMSFPQSAPHGVVFLHVTYVPAQEKNFTTAPAICHDGKAHFPREGVFVSNGTHWFVTQRNFYEPQIITTDNTFVSGNCDVVIGIVNNTVYDPLQPELDSFKEELDKYFKNHTSPDVDLGDISGINASVVNIQKEIDRLNEVAKNLNESLIDLQELGKYEQYIKWPWYIWLGFIAGLIAIVMVTIMLCCMTSCCSCLKGCCSCGSCC

SEQ ID NO: 41 - DNA, 3828 bp, synthetic construct
  misc_feature 1..3828: note = synthetic polynucleotide for Antigen_1_nCov_Spike_full_opt_h.sapiens_koz_2P
  source 1..3828: mol_type = other DNA
  CDS 7..3828
gccaccatgttcgtgtttctggtgctgctgcctctggtgtccagccagtgtgtgaacctgaccaccagaacacagctgcctccagcctacaccaacagctttaccagaggcgtgtactaccccgacaaggtgttcagatccagcgtgctgcactctacccaggacctgttcctgcctttcttcagcaacgtgacctggttccacgccatccacgtgtccggcaccaatggcaccaagagattcgacaaccccgtgctgcccttcaacgacggggtgtactttgccagcaccgagaagtccaacatcatcagaggctggatcttcggcaccacactggacagcaagacccagagcctgctgatcgtgaacaacgccaccaacgtggtcatcaaagtgtgcgagttccagttctgcaacgaccccttcctgggcgtctactaccacaagaacaacaagagctggatggaaagcgagttccgggtgtacagcagcgccaacaactgcaccttcgagtacgtgtcccagcctttcctgatggacctggaaggcaagcagggcaacttcaagaacctgcgcgagttcgtgttcaagaacatcgacggctacttcaagatctacagcaagcacacccctatcaacctcgtgcgggatctgcctcagggcttctctgctctggaacccctggtggatctgcccatcggcatcaacatcacccggtttcagacactgctggccctgcacagaagctacctgacacctggcgatagcagcagcggatggacagctggtgccgccgcttactatgtgggctacctgcagcctagaaccttcctgctgaagtacaacgagaacggcaccatcaccgacgccgtggattgtgctctggatcctctgagcgagacaaagtgcaccctgaagtccttcaccgtggaaaagggcatctaccagaccagcaacttccgggtgcagcccaccgaatccatcgtgcggttccccaatatcaccaatctgtgccccttcggcgaggtgttcaatgccaccagattcgcctctgtgtacgcctggaaccggaagcggatcagcaattgcgtggccgactactccgtgctgtacaactccgccagcttcagcaccttcaagtgctacggcgtgtcccctaccaagctgaacgacctgtgcttcacaaacgtgtacgccgacagcttcgtgatccggggagatgaagtgcggcagattgcccctggacagacaggcaagatcgccgactacaactacaagctgcccgacgacttcaccggctgtgtgattgcctggaacagcaacaacctggactccaaagtcggcggcaactacaattacctgtaccggctgttccggaagtccaatctgaagcccttcgagcgggacatctccaccgagatctatcaggccggcagcaccccttgtaacggcgtggaaggcttcaactgctacttcccactgcagtcctacggctttcagcccacaaatggcgtgggctatcagccctacagagtggtggtgctgagcttcgaactgctgcatgcccctgccacagtgtgcggccctaagaaaagcaccaatctcgtgaagaacaaatgcgtgaacttcaacttcaacggcctgaccggcaccggcgtgctgacagagagcaacaagaagttcctgccattccagcagtttggccgggatatcgccgataccacagacgccgttagagatccccagacactggaaatcctggacatcaccccttgcagcttcggcggagtgtctgtgatcacccctggcaccaacaccagcaatcaggtggcagtgctgtaccaggacgtgaactgtaccgaagtgcccgtggccattcacgccgatcagctgacacctacatggcgggtgtactccaccggcagcaatgtgtttcagaccagagccggctgtctgatcggagccgagcacgtgaacaatagctacgagtgcgacatccccatcggcgctggcatctgtgccagctaccagacacagacaaacagccccagacgggccagatctgtggccagccagagcatcattgcctacacaatgtctctgggcgccgagaacagcgtggcctactccaacaactctatcgctatccccaccaacttcaccatcagcgtgaccacagagatcctgcctgtgtccatgaccaagaccagcgtggactgcaccatgtacatctgcggcgattccaccgagtgctccaacctgctgctgcagtacggcagcttctgcacccagctgaatagagccctgacagggatcgccgtggaacaggacaagaacacccaagaggtgttcgcccaagtgaagcagatctacaagacccctcctatcaaggacttcggcggcttcaatttcagccagattctgcccgatcctagcaagcccagcaagcggagcttcatcgaggacctgctgttcaacaaagtgacactggccgacgccggcttcatcaagcagtatggcgattgtctgggcgacattgccgccagggatctgatttgcgcccagaagtttaacggactgacagtgctgcctcctctgctgaccgatgagatgatcgcccagtacacatctgccctgctggccggcacaatcacaagcggctggacatttggagctggcgccgctctgcagatcccctttgctatgcagatggcctaccggttcaacggcatcggagtgacccagaatgtgctgtacgagaaccagaagctgatcgccaaccagttcaacagcgccatcggcaagatccaggacagcctgagcagcacagcaagcgccctgggaaagctgcaggacgtggtcaaccagaatgcccaggcactgaacaccctggtcaagcagctgtcctccaacttcggcgccatcagctctgtgctgaacgatatcctgagcagactggacccgccggaagccgaggtgcagatcgacagactgatcaccggaaggctgcagtccctgcagacctacgttacccagcagctgatcagagccgccgagattagagcctctgccaatctggccgccaccaagatgtctgagtgtgtgctgggccagagcaagagagtggacttttgcggcaagggctaccacctgatgagcttccctcagtctgcccctcacggcgtggtgtttctgcacgtgacatacgtgcccgctcaagagaagaatttcaccaccgctccagccatctgccacgacggcaaagcccactttcctagagaaggcgtgttcgtgtccaacggcacccattggttcgtgacccagcggaacttctacgagccccagatcatcaccaccgacaacaccttcgtgtctggcaactgcgacgtcgtgatcggcattgtgaacaataccgtgtacgaccctctgcagcccgagctggacagcttcaaagaggaactggataagtactttaagaaccacacaagccccgacgtggacctgggcgatatcagcggaatcaatgccagcgtcgtgaacatccagaaagagatcgaccggctgaacgaggtggccaagaatctgaacgagagcctgatcgacctgcaagaactggggaagtacgagcagtacatcaagtggccctggtacatctggctgggctttatcgccggactgattgccatcgtgatggtcacaatcatgctgtgttgcatgaccagctgctgtagctgcctgaagggctgttgtagctgtggcagctgctgcaagttcgacgaggacgattctgagcccgtgctgaagggcgtgaaactgcactacacctga

SEQ ID NO: 42 - protein, 1273 aa, synthetic construct
  REGION 1..1273: note = Synthetic Construct
MFVFLVLLPLVSSQCVNLTTRTQLPPAYTNSFTRGVYYPDKVFRSSVLHSTQDLFLPFFSNVTWFHAIHVSGTNGTKRFDNPVLPFNDGVYFASTEKSNIIRGWIFGTTLDSKTQSLLIVNNATNVVIKVCEFQFCNDPFLGVYYHKNNKSWMESEFRVYSSANNCTFEYVSQPFLMDLEGKQGNFKNLREFVFKNIDGYFKIYSKHTPINLVRDLPQGFSALEPLVDLPIGINITRFQTLLALHRSYLTPGDSSSGWTAGAAAYYVGYLQPRTFLLKYNENGTITDAVDCALDPLSETKCTLKSFTVEKGIYQTSNFRVQPTESIVRFPNITNLCPFGEVFNATRFASVYAWNRKRISNCVADYSVLYNSASFSTFKCYGVSPTKLNDLCFTNVYADSFVIRGDEVRQIAPGQTGKIADYNYKLPDDFTGCVIAWNSNNLDSKVGGNYNYLYRLFRKSNLKPFERDISTEIYQAGSTPCNGVEGFNCYFPLQSYGFQPTNGVGYQPYRVVVLSFELLHAPATVCGPKKSTNLVKNKCVNFNFNGLTGTGVLTESNKKFLPFQQFGRDIADTTDAVRDPQTLEILDITPCSFGGVSVITPGTNTSNQVAVLYQDVNCTEVPVAIHADQLTPTWRVYSTGSNVFQTRAGCLIGAEHVNNSYECDIPIGAGICASYQTQTNSPRRARSVASQSIIAYTMSLGAENSVAYSNNSIAIPTNFTISVTTEILPVSMTKTSVDCTMYICGDSTECSNLLLQYGSFCTQLNRALTGIAVEQDKNTQEVFAQVKQIYKTPPIKDFGGFNFSQILPDPSKPSKRSFIEDLLFNKVTLADAGFIKQYGDCLGDIAARDLICAQKFNGLTVLPPLLTDEMIAQYTSALLAGTITSGWTFGAGAALQIPFAMQMAYRFNGIGVTQNVLYENQKLIANQFNSAIGKIQDSLSSTASALGKLQDVVNQNAQALNTLVKQLSSNFGAISSVLNDILSRLDPPEAEVQIDRLITGRLQSLQTYVTQQLIRAAEIRASANLAATKMSECVLGQSKRVDFCGKGYHLMSFPQSAPHGVVFLHVTYVPAQEKNFTTAPAICHDGKAHFPREGVFVSNGTHWFVTQRNFYEPQIITTDNTFVSGNCDVVIGIVNNTVYDPLQPELDSFKEELDKYFKNHTSPDVDLGDISGINASVVNIQKEIDRLNEVAKNLNESLIDLQELGKYEQYIKWPWYIWLGFIAGLIAIVMVTIMLCCMTSCCSCLKGCCSCGSCCKFDEDDSEPVLKGVKLHYT

SEQ ID NO: 43 - DNA, 3819 bp, synthetic construct
  misc_feature 1..3819: note = synthetic polynucleotide for Antigen_1_nCov_Spike_full_opt_h.sapiens_koz_UK
  source 1..3819: mol_type = other DNA
  CDS 7..3819
gccaccatgttcgtgtttctggtgctgctgcctctggtgtccagccagtgtgtgaacctgaccaccagaacacagctgcctccagcctacaccaacagctttaccagaggcgtgtactaccccgacaaggtgttcagatccagcgtgctgcactctacccaggacctgttcctgcctttcttcagcaacgtgacctggttccacgccatctccggcaccaatggcaccaagagattcgacaaccccgtgctgcccttcaacgacggggtgtactttgccagcaccgagaagtccaacatcatcagaggctggatcttcggcaccacactggacagcaagacccagagcctgctgatcgtgaacaacgccaccaacgtggtcatcaaagtgtgcgagttccagttctgcaacgaccccttcctgggcgtctaccacaagaacaacaagagctggatggaaagcgagttccgggtgtacagcagcgccaacaactgcaccttcgagtacgtgtcccagcctttcctgatggacctggaaggcaagcagggcaacttcaagaacctgcgcgagttcgtgttcaagaacatcgacggctacttcaagatctacagcaagcacacccctatcaacctcgtgcgggatctgcctcagggcttctctgctctggaacccctggtggatctgcccatcggcatcaacatcacccggtttcagacactgctggccctgcacagaagctacctgacacctggcgatagcagcagcggatggacagctggtgccgccgcttactatgtgggctacctgcagcctagaaccttcctgctgaagtacaacgagaacggcaccatcaccgacgccgtggattgtgctctggatcctctgagcgagacaaagtgcaccctgaagtccttcaccgtggaaaagggcatctaccagaccagcaacttccgggtgcagcccaccgaatccatcgtgcggttccccaatatcaccaatctgtgccccttcggcgaggtgttcaatgccaccagattcgcctctgtgtacgcctggaaccggaagcggatcagcaattgcgtggccgactactccgtgctgtacaactccgccagcttcagcaccttcaagtgctacggcgtgtcccctaccaagctgaacgacctgtgcttcacaaacgtgtacgccgacagcttcgtgatccggggagatgaagtgcggcagattgcccctggacagacaggcaagatcgccgactacaactacaagctgcccgacgacttcaccggctgtgtgattgcctggaacagcaacaacctggactccaaagtcggcggcaactacaattacctgtaccggctgttccggaagtccaatctgaagcccttcgagcgggacatctccaccgagatctatcaggccggcagcaccccttgtaacggcgtggaaggcttcaactgctacttcccactgcagtcctacggctttcagcccacatatggcgtgggctatcagccctacagagtggtggtgctgagcttcgaactgctgcatgcccctgccacagtgtgcggccctaagaaaagcaccaatctcgtgaagaacaaatgcgtgaacttcaacttcaacggcctgaccggcaccggcgtgctgacagagagcaacaagaagttcctgccattccagcagtttggccgggatatcgacgataccacagacgccgttagagatccccagacactggaaatcctggacatcaccccttgcagcttcggcggagtgtctgtgatcacccctggcaccaacaccagcaatcaggtggcagtgctgtaccagggcgtgaactgtaccgaagtgcccgtggccattcacgccgatcagctgacacctacatggcgggtgtactccaccggcagcaatgtgtttcagaccagagccggctgtctgatcggagccgagcacgtgaacaatagctacgagtgcgacatccccatcggcgctggcatctgtgccagctaccagacacagacaaacagccacagacgggccagatctgtggccagccagagcatcattgcctacacaatgtctctgggcgccgagaacagcgtggcctactccaacaactctatcgctatccccatcaacttcaccatcagcgtgaccacagagatcctgcctgtgtccatgaccaagaccagcgtggactgcaccatgtacatctgcggcgattccaccgagtgctccaacctgctgctgcagtacggcagcttctgcacccagctgaatagagccctgacagggatcgccgtggaacaggacaagaacacccaagaggtgttcgcccaagtgaagcagatctacaagacccctcctatcaaggacttcggcggcttcaatttcagccagattctgcccgatcctagcaagcccagcaagcggagcttcatcgaggacctgctgttcaacaaagtgacactggccgacgccggcttcatcaagcagtatggcgattgtctgggcgacattgccgccagggatctgatttgcgcccagaagtttaacggactgacagtgctgcctcctctgctgaccgatgagatgatcgcccagtacacatctgccctgctggccggcacaatcacaagcggctggacatttggagctggcgccgctctgcagatcccctttgctatgcagatggcctaccggttcaacggcatcggagtgacccagaatgtgctgtacgagaaccagaagctgatcgccaaccagttcaacagcgccatcggcaagatccaggacagcctgagcagcacagcaagcgccctgggaaagctgcaggacgtggtcaaccagaatgcccaggcactgaacaccctggtcaagcagctgtcctccaacttcggcgccatcagctctgtgctgaacgatatcctggccagactggacaaggtggaagccgaggtgcagatcgacagactgatcaccggaaggctgcagtccctgcagacctacgttacccagcagctgatcagagccgccgagattagagcctctgccaatctggccgccaccaagatgtctgagtgtgtgctgggccagagcaagagagtggacttttgcggcaagggctaccacctgatgagcttccctcagtctgcccctcacggcgtggtgtttctgcacgtgacatacgtgcccgctcaagagaagaatttcaccaccgctccagccatctgccacgacggcaaagcccactttcctagagaaggcgtgttcgtgtccaacggcacccattggttcgtgacccagcggaacttctacgagccccagatcatcaccacccacaacaccttcgtgtctggcaactgcgacgtcgtgatcggcattgtgaacaataccgtgtacgaccctctgcagcccgagctggacagcttcaaagaggaactggataagtactttaagaaccacacaagccccgacgtggacctgggcgatatcagcggaatcaatgccagcgtcgtgaacatccagaaagagatcgaccggctgaacgaggtggccaagaatctgaacgagagcctgatcgacctgcaagaactggggaagtacgagcagtacatcaagtggccctggtacatctggctgggctttatcgccggactgattgccatcgtgatggtcacaatcatgctgtgttgcatgaccagctgctgtagctgcctgaagggctgttgtagctgtggcagctgctgcaagttcgacgaggacgattctgagcccgtgctgaagggcgtgaaactgcactacacctga

SEQ ID NO: 44 - protein, 1270 aa, synthetic construct
  REGION 1..1270: note = Synthetic Construct
MFVFLVLLPLVSSQCVNLTTRTQLPPAYTNSFTRGVYYPDKVFRSSVLHSTQDLFLPFFSNVTWFHAISGTNGTKRFDNPVLPFNDGVYFASTEKSNIIRGWIFGTTLDSKTQSLLIVNNATNVVIKVCEFQFCNDPFLGVYHKNNKSWMESEFRVYSSANNCTFEYVSQPFLMDLEGKQGNFKNLREFVFKNIDGYFKIYSKHTPINLVRDLPQGFSALEPLVDLPIGINITRFQTLLALHRSYLTPGDSSSGWTAGAAAYYVGYLQPRTFLLKYNENGTITDAVDCALDPLSETKCTLKSFTVEKGIYQTSNFRVQPTESIVRFPNITNLCPFGEVFNATRFASVYAWNRKRISNCVADYSVLYNSASFSTFKCYGVSPTKLNDLCFTNVYADSFVIRGDEVRQIAPGQTGKIADYNYKLPDDFTGCVIAWNSNNLDSKVGGNYNYLYRLFRKSNLKPFERDISTEIYQAGSTPCNGVEGFNCYFPLQSYGFQPTYGVGYQPYRVVVLSFELLHAPATVCGPKKSTNLVKNKCVNFNFNGLTGTGVLTESNKKFLPFQQFGRDIDDTTDAVRDPQTLEILDITPCSFGGVSVITPGTNTSNQVAVLYQGVNCTEVPVAIHADQLTPTWRVYSTGSNVFQTRAGCLIGAEHVNNSYECDIPIGAGICASYQTQTNSHRRARSVASQSIIAYTMSLGAENSVAYSNNSIAIPINFTISVTTEILPVSMTKTSVDCTMYICGDSTECSNLLLQYGSFCTQLNRALTGIAVEQDKNTQEVFAQVKQIYKTPPIKDFGGFNFSQILPDPSKPSKRSFIEDLLFNKVTLADAGFIKQYGDCLGDIAARDLICAQKFNGLTVLPPLLTDEMIAQYTSALLAGTITSGWTFGAGAALQIPFAMQMAYRFNGIGVTQNVLYENQKLIANQFNSAIGKIQDSLSSTASALGKLQDVVNQNAQALNTLVKQLSSNFGAISSVLNDILARLDKVEAEVQIDRLITGRLQSLQTYVTQQLIRAAEIRASANLAATKMSECVLGQSKRVDFCGKGYHLMSFPQSAPHGVVFLHVTYVPAQEKNFTTAPAICHDGKAHFPREGVFVSNGTHWFVTQRNFYEPQIITTHNTFVSGNCDVVIGIVNNTVYDPLQPELDSFKEELDKYFKNHTSPDVDLGDISGINASVVNIQKEIDRLNEVAKNLNESLIDLQELGKYEQYIKWPWYIWLGFIAGLIAIVMVTIMLCCMTSCCSCLKGCCSCGSCCKFDEDDSEPVLKGVKLHYT

SEQ ID NO: 45 - DNA, 3762 bp, synthetic construct
  misc_feature 1..3762: note = synthetic polynucleotide for Antigen_1_nCov_Spike_full_opt_h.sapiens_koz_UK_delta_Cter
  source 1..3762: mol_type = other DNA
  CDS 7..3762
gccaccatgttcgtgtttctggtgctgctgcctctggtgtccagccagtgtgtgaacctgaccaccagaacacagctgcctccagcctacaccaacagctttaccagaggcgtgtactaccccgacaaggtgttcagatccagcgtgctgcactctacccaggacctgttcctgcctttcttcagcaacgtgacctggttccacgccatctccggcaccaatggcaccaagagattcgacaaccccgtgctgcccttcaacgacggggtgtactttgccagcaccgagaagtccaacatcatcagaggctggatcttcggcaccacactggacagcaagacccagagcctgctgatcgtgaacaacgccaccaacgtggtcatcaaagtgtgcgagttccagttctgcaacgaccccttcctgggcgtctaccacaagaacaacaagagctggatggaaagcgagttccgggtgtacagcagcgccaacaactgcaccttcgagtacgtgtcccagcctttcctgatggacctggaaggcaagcagggcaacttcaagaacctgcgcgagttcgtgttcaagaacatcgacggctacttcaagatctacagcaagcacacccctatcaacctcgtgcgggatctgcctcagggcttctctgctctggaacccctggtggatctgcccatcggcatcaacatcacccggtttcagacactgctggccctgcacagaagctacctgacacctggcgatagcagcagcggatggacagctggtgccgccgcttactatgtgggctacctgcagcctagaaccttcctgctgaagtacaacgagaacggcaccatcaccgacgccgtggattgtgctctggatcctctgagcgagacaaagtgcaccctgaagtccttcaccgtggaaaagggcatctaccagaccagcaacttccgggtgcagcccaccgaatccatcgtgcggttccccaatatcaccaatctgtgccccttcggcgaggtgttcaatgccaccagattcgcctctgtgtacgcctggaaccggaagcggatcagcaattgcgtggccgactactccgtgctgtacaactccgccagcttcagcaccttcaagtgctacggcgtgtcccctaccaagctgaacgacctgtgcttcacaaacgtgtacgccgacagcttcgtgatccggggagatgaagtgcggcagattgcccctggacagacaggcaagatcgccgactacaactacaagctgcccgacgacttcaccggctgtgtgattgcctggaacagcaacaacctggactccaaagtcggcggcaactacaattacctgtaccggctgttccggaagtccaatctgaagcccttcgagcgggacatctccaccgagatctatcaggccggcagcaccccttgtaacggcgtggaaggcttcaactgctacttcccactgcagtcctacggctttcagcccacatatggcgtgggctatcagccctacagagtggtggtgctgagcttcgaactgctgcatgcccctgccacagtgtgcggccctaagaaaagcaccaatctcgtgaagaacaaatgcgtgaacttcaacttcaacggcctgaccggcaccggcgtgctgacagagagcaacaagaagttcctgccattccagcagtttggccgggatatcgacgataccacagacgccgttagagatccccagacactggaaatcctggacatcaccccttgcagcttcggcggagtgtctgtgatcacccctggcaccaacaccagcaatcaggtggcagtgctgtaccagggcgtgaactgtaccgaagtgcccgtggccattcacgccgatcagctgacacctacatggcgggtgtactccaccggcagcaatgtgtttcagaccagagccggctgtctgatcggagccgagcacgtgaacaatagctacgagtgcgacatccccatcggcgctggcatctgtgccagctaccagacacagacaaacagccacagacgggccagatctgtggccagccagagcatcattgcctacacaatgtctctgggcgccgagaacagcgtggcctactccaacaactctatcgctatccccatcaacttcaccatcagcgtgaccacagagatcctgcctgtgtccatgaccaagaccagcgtggactgcaccatgtacatctgcggcgattccaccgagtgctccaacctgctgctgcagtacggcagcttctgcacccagctgaatagagccctgacagggatcgccgtggaacaggacaagaacacccaagaggtgttcgcccaagtgaagcagatctacaagacccctcctatcaaggacttcggcggcttcaatttcagccagattctgcccgatcctagcaagcccagcaagcggagcttcatcgaggacctgctgttcaacaaagtgacactggccgacgccggcttcatcaagcagtatggcgattgtctgggcgacattgccgccagggatctgatttgcgcccagaagtttaacggactgacagtgctgcctcctctgctgaccgatgagatgatcgcccagtacacatctgccctgctggccggcacaatcacaagcggctggacatttggagctggcgccgctctgcagatcccctttgctatgcagatggcctaccggttcaacggcatcggagtgacccagaatgtgctgtacgagaaccagaagctgatcgccaaccagttcaacagcgccatcggcaagatccaggacagcctgagcagcacagcaagcgccctgggaaagctgcaggacgtggtcaaccagaatgcccaggcactgaacaccctggtcaagcagctgtcctccaacttcggcgccatcagctctgtgctgaacgatatcctggccagactggacaaggtggaagccgaggtgcagatcgacagactgatcaccggaaggctgcagtccctgcagacctacgttacccagcagctgatcagagccgccgagattagagcctctgccaatctggccgccaccaagatgtctgagtgtgtgctgggccagagcaagagagtggacttttgcggcaagggctaccacctgatgagcttccctcagtctgcccctcacggcgtggtgtttctgcacgtgacatacgtgcccgctcaagagaagaatttcaccaccgctccagccatctgccacgacggcaaagcccactttcctagagaaggcgtgttcgtgtccaacggcacccattggttcgtgacccagcggaacttctacgagccccagatcatcaccacccacaacaccttcgtgtctggcaactgcgacgtcgtgatcggcattgtgaacaataccgtgtacgaccctctgcagcccgagctggacagcttcaaagaggaactggataagtactttaagaaccacacaagccccgacgtggacctgggcgatatcagcggaatcaatgccagcgtcgtgaacatccagaaagagatcgaccggctgaacgaggtggccaagaatctgaacgagagcctgatcgacctgcaagaactggggaagtacgagcagtacatcaagtggccctggtacatctggctgggctttatcgccggactgattgccatcgtgatggtcacaatcatgctgtgttgcatgaccagctgctgtagctgcctgaagggctgttgtagctgtggcagctgctgctga

SEQ ID NO: 46 - protein, 1251 aa, synthetic construct
  REGION 1..1251: note = Synthetic Construct
MFVFLVLLPLVSSQCVNLTTRTQLPPAYTNSFTRGVYYPDKVFRSSVLHSTQDLFLPFFSNVTWFHAISGTNGTKRFDNPVLPFNDGVYFASTEKSNIIRGWIFGTTLDSKTQSLLIVNNATNVVIKVCEFQFCNDPFLGVYHKNNKSWMESEFRVYSSANNCTFEYVSQPFLMDLEGKQGNFKNLREFVFKNIDGYFKIYSKHTPINLVRDLPQGFSALEPLVDLPIGINITRFQTLLALHRSYLTPGDSSSGWTAGAAAYYVGYLQPRTFLLKYNENGTITDAVDCALDPLSETKCTLKSFTVEKGIYQTSNFRVQPTESIVRFPNITNLCPFGEVFNATRFASVYAWNRKRISNCVADYSVLYNSASFSTFKCYGVSPTKLNDLCFTNVYADSFVIRGDEVRQIAPGQTGKIADYNYKLPDDFTGCVIAWNSNNLDSKVGGNYNYLYRLFRKSNLKPFERDISTEIYQAGSTPCNGVEGFNCYFPLQSYGFQPTYGVGYQPYRVVVLSFELLHAPATVCGPKKSTNLVKNKCVNFNFNGLTGTGVLTESNKKFLPFQQFGRDIDDTTDAVRDPQTLEILDITPCSFGGVSVITPGTNTSNQVAVLYQGVNCTEVPVAIHADQLTPTWRVYSTGSNVFQTRAGCLIGAEHVNNSYECDIPIGAGICASYQTQTNSHRRARSVASQSIIAYTMSLGAENSVAYSNNSIAIPINFTISVTTEILPVSMTKTSVDCTMYICGDSTECSNLLLQYGSFCTQLNRALTGIAVEQDKNTQEVFAQVKQIYKTPPIKDFGGFNFSQILPDPSKPSKRSFIEDLLFNKVTLADAGFIKQYGDCLGDIAARDLICAQKFNGLTVLPPLLTDEMIAQYTSALLAGTITSGWTFGAGAALQIPFAMQMAYRFNGIGVTQNVLYENQKLIANQFNSAIGKIQDSLSSTASALGKLQDVVNQNAQALNTLVKQLSSNFGAISSVLNDILARLDKVEAEVQIDRLITGRLQSLQTYVTQQLIRAAEIRASANLAATKMSECVLGQSKRVDFCGKGYHLMSFPQSAPHGVVFLHVTYVPAQEKNFTTAPAICHDGKAHFPREGVFVSNGTHWFVTQRNFYEPQIITTHNTFVSGNCDVVIGIVNNTVYDPLQPELDSFKEELDKYFKNHTSPDVDLGDISGINASVVNIQKEIDRLNEVAKNLNESLIDLQELGKYEQYIKWPWYIWLGFIAGLIAIVMVTIMLCCMTSCCSCLKGCCSCGSCC

SEQ ID NO: 47 - DNA, 3819 bp, synthetic construct
  misc_feature 1..3819: note = synthetic polynucleotide for Antigen_1_nCov_Spike_full_opt_h.sapiens_koz_UK_2P
  source 1..3819: mol_type = other DNA
  CDS 7..3819
gccaccatgttcgtgtttctggtgctgctgcctctggtgtccagccagtgtgtgaacctgaccaccagaacacagctgcctccagcctacaccaacagctttaccagaggcgtgtactaccccgacaaggtgttcagatccagcgtgctgcactctacccaggacctgttcctgcctttcttcagcaacgtgacctggttccacgccatctccggcaccaatggcaccaagagattcgacaaccccgtgctgcccttcaacgacggggtgtactttgccagcaccgagaagtccaacatcatcagaggctggatcttcggcaccacactggacagcaagacccagagcctgctgatcgtgaacaacgccaccaacgtggtcatcaaagtgtgcgagttccagttctgcaacgaccccttcctgggcgtctaccacaagaacaacaagagctggatggaaagcgagttccgggtgtacagcagcgccaacaactgcaccttcgagtacgtgtcccagcctttcctgatggacctggaaggcaagcagggcaacttcaagaacctgcgcgagttcgtgttcaagaacatcgacggctacttcaagatctacagcaagcacacccctatcaacctcgtgcgggatctgcctcagggcttctctgctctggaacccctggtggatctgcccatcggcatcaacatcacccggtttcagacactgctggccctgcacagaagctacctgacacctggcgatagcagcagcggatggacagctggtgccgccgcttactatgtgggctacctgcagcctagaaccttcctgctgaagtacaacgagaacggcaccatcaccgacgccgtggattgtgctctggatcctctgagcgagacaaagtgcaccctgaagtccttcaccgtggaaaagggcatctaccagaccagcaacttccgggtgcagcccaccgaatccatcgtgcggttccccaatatcaccaatctgtgccccttcggcgaggtgttcaatgccaccagattcgcctctgtgtacgcctggaaccggaagcggatcagcaattgcgtggccgactactccgtgctgtacaactccgccagcttcagcaccttcaagtgctacggcgtgtcccctaccaagctgaacgacctgtgcttcacaaacgtgtacgccgacagcttcgtgatccggggagatgaagtgcggcagattgcccctggacagacaggcaagatcgccgactacaactacaagctgcccgacgacttcaccggctgtgtgattgcctggaacagcaacaacctggactccaaagtcggcggcaactacaattacctgtaccggctgttccggaagtccaatctgaagcccttcgagcgggacatctccaccgagatctatcaggccggcagcaccccttgtaacggcgtggaaggcttcaactgctacttcccactgcagtcctacggctttcagcccacatatggcgtgggctatcagccctacagagtggtggtgctgagcttcgaactgctgcatgcccctgccacagtgtgcggccctaagaaaagcaccaatctcgtgaagaacaaatgcgtgaacttcaacttcaacggcctgaccggcaccggcgtgctgacagagagcaacaagaagttcctgccattccagcagtttggccgggatatcgacgataccacagacgccgttagagatccccagacactggaaatcctggacatcaccccttgcagcttcggcggagtgtctgtgatcacccctggcaccaacaccagcaatcaggtggcagtgctgtaccagggcgtgaactgtaccgaagtgcccgtggccattcacgccgatcagctgacacctacatggcgggtgtactccaccggcagcaatgtgtttcagaccagagccggctgtctgatcggagccgagcacgtgaacaatagctacgagtgcgacatccccatcggcgctggcatctgtgccagctaccagacacagacaaacagccacagacgggccagatctgtggccagccagagcatcattgcctacacaatgtctctgggcgccgagaacagcgtggcctactccaacaactctatcgctatccccatcaacttcaccatcagcgtgaccacagagatcctgcctgtgtccatgaccaagaccagcgtggactgcaccatgtacatctgcggcgattccaccgagtgctccaacctgctgctgcagtacggcagcttctgcacccagctgaatagagccctgacagggatcgccgtggaacaggacaagaacacccaagaggtgttcgcccaagtgaagcagatctacaagacccctcctatcaaggacttcggcggcttcaatttcagccagattctgcccgatcctagcaagcccagcaagcggagcttcatcgaggacctgctgttcaacaaagtgacactggccgacgccggcttcatcaagcagtatggcgattgtctgggcgacattgccgccagggatctgatttgcgcccagaagtttaacggactgacagtgctgcctcctctgctgaccgatgagatgatcgcccagtacacatctgccctgctggccggcacaatcacaagcggctggacatttggagctggcgccgctctgcagatcccctttgctatgcagatggcctaccggttcaacggcatcggagtgacccagaatgtgctgtacgagaaccagaagctgatcgccaaccagttcaacagcgccatcggcaagatccaggacagcctgagcagcacagcaagcgccctgggaaagctgcaggacgtggtcaaccagaatgcccaggcactgaacaccctggtcaagcagctgtcctccaacttcggcgccatcagctctgtgctgaacgatatcctggccagactggacccgccggaagccgaggtgcagatcgacagactgatcaccggaaggctgcagtccctgcagacctacgttacccagcagctgatcagagccgccgagattagagcctctgccaatctggccgccaccaagatgtctgagtgtgtgctgggccagagcaagagagtggacttttgcggcaagggctaccacctgatgagcttccctcagtctgcccctcacggcgtggtgtttctgcacgtgacatacgtgcccgctcaagagaagaatttcaccaccgctccagccatctgccacgacggcaaagcccactttcctagagaaggcgtgttcgtgtccaacggcacccattggttcgtgacccagcggaacttctacgagccccagatcatcaccacccacaacaccttcgtgtctggcaactgcgacgtcgtgatcggcattgtgaacaataccgtgtacgaccctctgcagcccgagctggacagcttcaaagaggaactggataagtactttaagaaccacacaagccccgacgtggacctgggcgatatcagcggaatcaatgccagcgtcgtgaacatccagaaagagatcgaccggctgaacgaggtggccaagaatctgaacgagagcctgatcgacctgcaagaactggggaagtacgagcagtacatcaagtggccctggtacatctggctgggctttatcgccggactgattgccatcgtgatggtcacaatcatgctgtgttgcatgaccagctgctgtagctgcctgaagggctgttgtagctgtggcagctgctgcaagttcgacgaggacgattctgagcccgtgctgaagggcgtgaaactgcactacacctga

SEQ ID NO: 48 - protein, 1270 aa, synthetic construct
  REGION 1..1270: note = Synthetic Construct
MFVFLVLLPLVSSQCVNLTTRTQLPPAYTNSFTRGVYYPDKVFRSSVLHSTQDLFLPFFSNVTWFHAISGTNGTKRFDNPVLPFNDGVYFASTEKSNIIRGWIFGTTLDSKTQSLLIVNNATNVVIKVCEFQFCNDPFLGVYHKNNKSWMESEFRVYSSANNCTFEYVSQPFLMDLEGKQGNFKNLREFVFKNIDGYFKIYSKHTPINLVRDLPQGFSALEPLVDLPIGINITRFQTLLALHRSYLTPGDSSSGWTAGAAAYYVGYLQPRTFLLKYNENGTITDAVDCALDPLSETKCTLKSFTVEKGIYQTSNFRVQPTESIVRFPNITNLCPFGEVFNATRFASVYAWNRKRISNCVADYSVLYNSASFSTFKCYGVSPTKLNDLCFTNVYADSFVIRGDEVRQIAPGQTGKIADYNYKLPDDFTGCVIAWNSNNLDSKVGGNYNYLYRLFRKSNLKPFERDISTEIYQAGSTPCNGVEGFNCYFPLQSYGFQPTYGVGYQPYRVVVLSFELLHAPATVCGPKKSTNLVKNKCVNFNFNGLTGTGVLTESNKKFLPFQQFGRDIDDTTDAVRDPQTLEILDITPCSFGGVSVITPGTNTSNQVAVLYQGVNCTEVPVAIHADQLTPTWRVYSTGSNVFQTRAGCLIGAEHVNNSYECDIPIGAGICASYQTQTNSHRRARSVASQSIIAYTMSLGAENSVAYSNNSIAIPINFTISVTTEILPVSMTKTSVDCTMYICGDSTECSNLLLQYGSFCTQLNRALTGIAVEQDKNTQEVFAQVKQIYKTPPIKDFGGFNFSQILPDPSKPSKRSFIEDLLFNKVTLADAGFIKQYGDCLGDIAARDLICAQKFNGLTVLPPLLTDEMIAQYTSALLAGTITSGWTFGAGAALQIPFAMQMAYRFNGIGVTQNVLYENQKLIANQFNSAIGKIQDSLSSTASALGKLQDVVNQNAQALNTLVKQLSSNFGAISSVLNDILARLDPPEAEVQIDRLITGRLQSLQTYVTQQLIRAAEIRASANLAATKMSECVLGQSKRVDFCGKGYHLMSFPQSAPHGVVFLHVTYVPAQEKNFTTAPAICHDGKAHFPREGVFVSNGTHWFVTQRNFYEPQIITTHNTFVSGNCDVVIGIVNNTVYDPLQPELDSFKEELDKYFKNHTSPDVDLGDISGINASVVNIQKEIDRLNEVAKNLNESLIDLQELGKYEQYIKWPWYIWLGFIAGLIAIVMVTIMLCCMTSCCSCLKGCCSCGSCCKFDEDDSEPVLKGVKLHYT

SEQ ID NO: 49 - DNA, 3762 bp, synthetic construct
  misc_feature 1..3762: note = synthetic polynucleotide for Antigen_1_nCov_Spike_full_opt_h.sapiens_koz_UK_2P_delta_Cter
  source 1..3762: mol_type = other DNA
  CDS 7..3762
gccaccatgttcgtgtttctggtgctgctgcctctggtgtccagccagtgtgtgaacctgaccaccagaacacagctgcctccagcctacaccaacagctttaccagaggcgtgtactaccccgacaaggtgttcagatccagcgtgctgcactctacccaggacctgttcctgcctttcttcagcaacgtgacctggttccacgccatctccggcaccaatggcaccaagagattcgacaaccccgtgctgcccttcaacgacggggtgtactttgccagcaccgagaagtccaacatcatcagaggctggatcttcggcaccacactggacagcaagacccagagcctgctgatcgtgaacaacgccaccaacgtggtcatcaaagtgtgcgagttccagttctgcaacgaccccttcctgggcgtctaccacaagaacaacaagagctggatggaaagcgagttccgggtgtacagcagcgccaacaactgcaccttcgagtacgtgtcccagcctttcctgatggacctggaaggcaagcagggcaacttcaagaacctgcgcgagttcgtgttcaagaacatcgacggctacttcaagatctacagcaagcacacccctatcaacctcgtgcgggatctgcctcagggcttctctgctctggaacccctggtggatctgcccatcggcatcaacatcacccggtttcagacactgctggccctgcacagaagctacctgacacctggcgatagcagcagcggatggacagctggtgccgccgcttactatgtgggctacctgcagcctagaaccttcctgctgaagtacaacgagaacggcaccatcaccgacgccgtggattgtgctctggatcctctgagcgagacaaagtgcaccctgaagtccttcaccgtggaaaagggcatctaccagaccagcaacttccgggtgcagcccaccgaatccatcgtgcggttccccaatatcaccaatctgtgccccttcggcgaggtgttcaatgccaccagattcgcctctgtgtacgcctggaaccggaagcggatcagcaattgcgtggccgactactccgtgctgtacaactccgccagcttcagcaccttcaagtgctacggcgtgtcccctaccaagctgaacgacctgtgcttcacaaacgtgtacgccgacagcttcgtgatccggggagatgaagtgcggcagattgcccctggacagacaggcaagatcgccgactacaactacaagctgcccgacgacttcaccggctgtgtgattgcctggaacagcaacaacctggactccaaagtcggcggcaactacaattacctgtaccggctgttccggaagtccaatctgaagcccttcgagcgggacatctccaccgagatctatcaggccggcagcaccccttgtaacggcgtggaaggcttcaactgctacttcccactgcagtcctacggctttcagcccacatatggcgtgggctatcagccctacagagtggtggtgctgagcttcgaactgctgcatgcccctgccacagtgtgcggccctaagaaaagcaccaatctcgtgaagaacaaatgcgtgaacttcaacttcaacggcctgaccggcaccggcgtgctgacagagagcaacaagaagttcctgccattccagcagtttggccgggatatcgacgataccacagacgccgttagagatccccagacactggaaatcctggacatcaccccttgcagcttcggcggagtgtctgtgatcacccctggcaccaacaccagcaatcaggtggcagtgctgtaccagggcgtgaactgtaccgaagtgcccgtggccattcacgccgatcagctgacacctacatggcgggtgtactccaccggcagcaatgtgtttcagaccagagccggctgtctgatcggagccgagcacgtgaacaatagctacgagtgcgacatccccatcggcgctggcatctgtgccagctaccagacacagacaaacagccacagacgggccagatctgtggccagccagagcatcattgcctacacaatgtctctgggcgccgagaacagcgtggcctactccaacaactctatcgctatccccatcaacttcaccatcagcgtgaccacagagatcctgcctgtgtccatgaccaagaccagcgtggactgcaccatgtacatctgcggcgattccaccgagtgctccaacctgctgctgcagtacggcagcttctgcacccagctgaatagagccctgacagggatcgccgtggaacaggacaagaacacccaagaggtgttcgcccaagtgaagcagatctacaagacccctcctatcaaggacttcggcggcttcaatttcagccagattctgcccgatcctagcaagcccagcaagcggagcttcatcgaggacctgctgttcaacaaagtgacactggccgacgccggcttcatcaagcagtatggcgattgtctgggcgacattgccgccagggatctgatttgcgcccagaagtttaacggactgacagtgctgcctcctctgctgaccgatgagatgatcgcccagtacacatctgccctgctggccggcacaatcacaagcggctggacatttggagctggcgccgctctgcagatcccctttgctatgcagatggcctaccggttcaacggcatcggagtgacccagaatgtgctgtacgagaaccagaagctgatcgccaaccagttcaacagcgccatcggcaagatccaggacagcctgagcagcacagcaagcgccctgggaaagctgcaggacgtggtcaaccagaatgcccaggcactgaacaccctggtcaagcagctgtcctccaacttcggcgccatcagctctgtgctgaacgatatcctggccagactggacccgccggaagccgaggtgcagatcgacagactgatcaccggaaggctgcagtccctgcagacctacgttacccagcagctgatcagagccgccgagattagagcctctgccaatctggccgccaccaagatgtctgagtgtgtgctgggccagagcaagagagtggacttttgcggcaagggctaccacctgatgagcttccctcagtctgcccctcacggcgtggtgtttctgcacgtgacatacgtgcccgctcaagagaagaatttcaccaccgctccagccatctgccacgacggcaaagcccactttcctagagaaggcgtgttcgtgtccaacggcacccattggttcgtgacccagcggaacttctacgagccccagatcatcaccacccacaacaccttcgtgtctggcaactgcgacgtcgtgatcggcattgtgaacaataccgtgtacgaccctctgcagcccgagctggacagcttcaaagaggaactggataagtactttaagaaccacacaagccccgacgtggacctgggcgatatcagcggaatcaatgccagcgtcgtgaacatccagaaagagatcgaccggctgaacgaggtggccaagaatctgaacgagagcctgatcgacctgcaagaactggggaagtacgagcagtacatcaagtggccctggtacatctggctgggctttatcgccggactgattgccatcgtgatggtcacaatcatgctgtgttgcatgaccagctgctgtagctgcctgaagggctgttgtagctgtggcagctgctgctga

SEQ ID NO: 50 - protein, 1251 aa, synthetic construct
  REGION 1..1251: note = Synthetic Construct
MFVFLVLLPLVSSQCVNLTTRTQLPPAYTNSFTRGVYYPDKVFRSSVLHSTQDLFLPFFSNVTWFHAISGTNGTKRFDNPVLPFNDGVYFASTEKSNIIRGWIFGTTLDSKTQSLLIVNNATNVVIKVCEFQFCNDPFLGVYHKNNKSWMESEFRVYSSANNCTFEYVSQPFLMDLEGKQGNFKNLREFVFKNIDGYFKIYSKHTPINLVRDLPQGFSALEPLVDLPIGINITRFQTLLALHRSYLTPGDSSSGWTAGAAAYYVGYLQPRTFLLKYNENGTITDAVDCALDPLSETKCTLKSFTVEKGIYQTSNFRVQPTESIVRFPNITNLCPFGEVFNATRFASVYAWNRKRISNCVADYSVLYNSASFSTFKCYGVSPTKLNDLCFTNVYADSFVIRGDEVRQIAPGQTGKIADYNYKLPDDFTGCVIAWNSNNLDSKVGGNYNYLYRLFRKSNLKPFERDISTEIYQAGSTPCNGVEGFNCYFPLQSYGFQPTYGVGYQPYRVVVLSFELLHAPATVCGPKKSTNLVKNKCVNFNFNGLTGTGVLTESNKKFLPFQQFGRDIDDTTDAVRDPQTLEILDITPCSFGGVSVITPGTNTSNQVAVLYQGVNCTEVPVAIHADQLTPTWRVYSTGSNVFQTRAGCLIGAEHVNNSYECDIPIGAGICASYQTQTNSHRRARSVASQSIIAYTMSLGAENSVAYSNNSIAIPINFTISVTTEILPVSMTKTSVDCTMYICGDSTECSNLLLQYGSFCTQLNRALTGIAVEQDKNTQEVFAQVKQIYKTPPIKDFGGFNFSQILPDPSKPSKRSFIEDLLFNKVTLADAGFIKQYGDCLGDIAARDLICAQKFNGLTVLPPLLTDEMIAQYTSALLAGTITSGWTFGAGAALQIPFAMQMAYRFNGIGVTQNVLYENQKLIANQFNSAIGKIQDSLSSTASALGKLQDVVNQNAQALNTLVKQLSSNFGAISSVLNDILARLDPPEAEVQIDRLITGRLQSLQTYVTQQLIRAAEIRASANLAATKMSECVLGQSKRVDFCGKGYHLMSFPQSAPHGVVFLHVTYVPAQEKNFTTAPAICHDGKAHFPREGVFVSNGTHWFVTQRNFYEPQIITTHNTFVSGNCDVVIGIVNNTVYDPLQPELDSFKEELDKYFKNHTSPDVDLGDISGINASVVNIQKEIDRLNEVAKNLNESLIDLQELGKYEQYIKWPWYIWLGFIAGLIAIVMVTIMLCCMTSCCSCLKGCCSCGSCC

SEQ ID NO: 51 - DNA, 3819 bp, synthetic construct
  misc_feature 1..3819: note = synthtic polynucleotide for Antigen_1_nCov_Spike_full_opt_h.sapiens_koz_SA
  source 1..3819: mol_type = other DNA
  CDS 7..3819
gccaccatgttcgtgtttctggtgctgctgcctctggtgtccagccagtgtgtgaactttaccaccagaacacagctgcctccagcctacaccaacagctttaccagaggcgtgtactaccccgacaaggtgttcagatccagcgtgctgcactctacccaggacctgttcctgcctttcttcagcaacgtgacctggttccacgccatccacgtgtccggcaccaatggcaccaagagattcgccaaccccgtgctgcccttcaacgacggggtgtactttgccagcaccgagaagtccaacatcatcagaggctggatcttcggcaccacactggacagcaagacccagagcctgctgatcgtgaacaacgccaccaacgtggtcatcaaagtgtgcgagttccagttctgcaacgaccccttcctgggcgtctactaccacaagaacaacaagagctggatggaaagcgagttccgggtgtacagcagcgccaacaactgcaccttcgagtacgtgtcccagcctttcctgatggacctggaaggcaagcagggcaacttcaagaacctgcgcgagttcgtgttcaagaacatcgacggctacttcaagatctacagcaagcacacccctatcaacctcgtgcggggtctgcctcagggcttctctgctctggaacccctggtggatctgcccatcggcatcaacatcacccggtttcagaccctgcacagaagctacctgacacctggcgatagcagcagcggatggacagctggtgccgccgcttactatgtgggctacctgcagcctagaaccttcctgctgaagtacaacgagaacggcaccatcaccgacgccgtggattgtgctctggatcctctgagcgagacaaagtgcaccctgaagtccttcaccgtggaaaagggcatctaccagaccagcaacttccgggtgcagcccaccgaatccatcgtgcggttccccaatatcaccaatctgtgccccttcggcgaggtgttcaatgccaccagattcgcctctgtgtacgcctggaaccggaagcggatcagcaattgcgtggccgactactccgtgctgtacaactccgccagcttcagcaccttcaagtgctacggcgtgtcccctaccaagctgaacgacctgtgcttcacaaacgtgtacgccgacagcttcgtgatccggggagatgaagtgcggcagattgcccctggacagacaggcaatatcgccgactacaactacaagctgcccgacgacttcaccggctgtgtgattgcctggaacagcaacaacctggactccaaagtcggcggcaactacaattacctgtaccggctgttccggaagtccaatctgaagcccttcgagcgggacatctccaccgagatctatcaggccggcagcaccccttgtaacggcgtgaaaggcttcaactgctacttcccactgcagtcctacggctttcagcccacatatggcgtgggctatcagccctacagagtggtggtgctgagcttcgaactgctgcatgcccctgccacagtgtgcggccctaagaaaagcaccaatctcgtgaagaacaaatgcgtgaacttcaacttcaacggcctgaccggcaccggcgtgctgacagagagcaacaagaagttcctgccattccagcagtttggccgggatatcgccgataccacagacgccgttagagatccccagacactggaaatcctggacatcaccccttgcagcttcggcggagtgtctgtgatcacccctggcaccaacaccagcaatcaggtggcagtgctgtaccagggcgtgaactgtaccgaagtgcccgtggccattcacgccgatcagctgacacctacatggcgggtgtactccaccggcagcaatgtgtttcagaccagagccggctgtctgatcggagccgagcacgtgaacaatagctacgagtgcgacatccccatcggcgctggcatctgtgccagctaccagacacagacaaacagccccagacgggccagatctgtggccagccagagcatcattgcctacacaatgtctctgggcgtcgagaacagcgtggcctactccaacaactctatcgctatccccaccaacttcaccatcagcgtgaccacagagatcctgcctgtgtccatgaccaagaccagcgtggactgcaccatgtacatctgcggcgattccaccgagtgctccaacctgctgctgcagtacggcagcttctgcacccagctgaatagagccctgacagggatcgccgtggaacaggacaagaacacccaagaggtgttcgcccaagtgaagcagatctacaagacccctcctatcaaggacttcggcggcttcaatttcagccagattctgcccgatcctagcaagcccagcaagcggagcttcatcgaggacctgctgttcaacaaagtgacactggccgacgccggcttcatcaagcagtatggcgattgtctgggcgacattgccgccagggatctgatttgcgcccagaagtttaacggactgacagtgctgcctcctctgctgaccgatgagatgatcgcccagtacacatctgccctgctggccggcacaatcacaagcggctggacatttggagctggcgccgctctgcagatcccctttgctatgcagatggcctaccggttcaacggcatcggagtgacccagaatgtgctgtacgagaaccagaagctgatcgccaaccagttcaacagcgccatcggcaagatccaggacagcctgagcagcacagcaagcgccctgggaaagctgcaggacgtggtcaaccagaatgcccaggcactgaacaccctggtcaagcagctgtcctccaacttcggcgccatcagctctgtgctgaacgatatcctgagcagactggacaaggtggaagccgaggtgcagatcgacagactgatcaccggaaggctgcagtccctgcagacctacgttacccagcagctgatcagagccgccgagattagagcctctgccaatctggccgccaccaagatgtctgagtgtgtgctgggccagagcaagagagtggacttttgcggcaagggctaccacctgatgagcttccctcagtctgcccctcacggcgtggtgtttctgcacgtgacatacgtgcccgctcaagagaagaatttcaccaccgctccagccatctgccacgacggcaaagcccactttcctagagaaggcgtgttcgtgtccaacggcacccattggttcgtgacccagcggaacttctacgagccccagatcatcaccaccgacaacaccttcgtgtctggcaactgcgacgtcgtgatcggcattgtgaacaataccgtgtacgaccctctgcagcccgagctggacagcttcaaagaggaactggataagtactttaagaaccacacaagccccgacgtggacctgggcgatatcagcggaatcaatgccagcgtcgtgaacatccagaaagagatcgaccggctgaacgaggtggccaagaatctgaacgagagcctgatcgacctgcaagaactggggaagtacgagcagtacatcaagtggccctggtacatctggctgggctttatcgccggactgattgccatcgtgatggtcacaatcatgctgtgttgcatgaccagctgctgtagctgcctgaagggctgttgtagctgtggcagctgctgcaagttcgacgaggacgattctgagcccgtgctgaagggcgtgaaactgcactacacctga

SEQ ID NO: 52 - protein, 1270 aa, synthetic construct
  REGION 1..1270: note = Synthetic Construct
MFVFLVLLPLVSSQCVNFTTRTQLPPAYTNSFTRGVYYPDKVFRSSVLHSTQDLFLPFFSNVTWFHAIHVSGTNGTKRFANPVLPFNDGVYFASTEKSNIIRGWIFGTTLDSKTQSLLIVNNATNVVIKVCEFQFCNDPFLGVYYHKNNKSWMESEFRVYSSANNCTFEYVSQPFLMDLEGKQGNFKNLREFVFKNIDGYFKIYSKHTPINLVRGLPQGFSALEPLVDLPIGINITRFQTLHRSYLTPGDSSSGWTAGAAAYYVGYLQPRTFLLKYNENGTITDAVDCALDPLSETKCTLKSFTVEKGIYQTSNFRVQPTESIVRFPNITNLCPFGEVFNATRFASVYAWNRKRISNCVADYSVLYNSASFSTFKCYGVSPTKLNDLCFTNVYADSFVIRGDEVRQIAPGQTGNIADYNYKLPDDFTGCVIAWNSNNLDSKVGGNYNYLYRLFRKSNLKPFERDISTEIYQAGSTPCNGVKGFNCYFPLQSYGFQPTYGVGYQPYRVVVLSFELLHAPATVCGPKKSTNLVKNKCVNFNFNGLTGTGVLTESNKKFLPFQQFGRDIADTTDAVRDPQTLEILDITPCSFGGVSVITPGTNTSNQVAVLYQGVNCTEVPVAIHADQLTPTWRVYSTGSNVFQTRAGCLIGAEHVNNSYECDIPIGAGICASYQTQTNSPRRARSVASQSIIAYTMSLGVENSVAYSNNSIAIPTNFTISVTTEILPVSMTKTSVDCTMYICGDSTECSNLLLQYGSFCTQLNRALTGIAVEQDKNTQEVFAQVKQIYKTPPIKDFGGFNFSQILPDPSKPSKRSFIEDLLFNKVTLADAGFIKQYGDCLGDIAARDLICAQKFNGLTVLPPLLTDEMIAQYTSALLAGTITSGWTFGAGAALQIPFAMQMAYRFNGIGVTQNVLYENQKLIANQFNSAIGKIQDSLSSTASALGKLQDVVNQNAQALNTLVKQLSSNFGAISSVLNDILSRLDKVEAEVQIDRLITGRLQSLQTYVTQQLIRAAEIRASANLAATKMSECVLGQSKRVDFCGKGYHLMSFPQSAPHGVVFLHVTYVPAQEKNFTTAPAICHDGKAHFPREGVFVSNGTHWFVTQRNFYEPQIITTDNTFVSGNCDVVIGIVNNTVYDPLQPELDSFKEELDKYFKNHTSPDVDLGDISGINASVVNIQKEIDRLNEVAKNLNESLIDLQELGKYEQYIKWPWYIWLGFIAGLIAIVMVTIMLCCMTSCCSCLKGCCSCGSCCKFDEDDSEPVLKGVKLHYT

SEQ ID NO: 53 - DNA, 3762 bp, synthetic construct
  misc_feature 1..3762: note = synthetic polynucleotide for Antigen_1_nCov_Spike_full_opt_h.sapiens_koz_SA_delta_Cter
  source 1..3762: mol_type = other DNA
  CDS 7..3762
gccaccatgttcgtgtttctggtgctgctgcctctggtgtccagccagtgtgtgaactttaccaccagaacacagctgcctccagcctacaccaacagctttaccagaggcgtgtactaccccgacaaggtgttcagatccagcgtgctgcactctacccaggacctgttcctgcctttcttcagcaacgtgacctggttccacgccatccacgtgtccggcaccaatggcaccaagagattcgccaaccccgtgctgcccttcaacgacggggtgtactttgccagcaccgagaagtccaacatcatcagaggctggatcttcggcaccacactggacagcaagacccagagcctgctgatcgtgaacaacgccaccaacgtggtcatcaaagtgtgcgagttccagttctgcaacgaccccttcctgggcgtctactaccacaagaacaacaagagctggatggaaagcgagttccgggtgtacagcagcgccaacaactgcaccttcgagtacgtgtcccagcctttcctgatggacctggaaggcaagcagggcaacttcaagaacctgcgcgagttcgtgttcaagaacatcgacggctacttcaagatctacagcaagcacacccctatcaacctcgtgcggggtctgcctcagggcttctctgctctggaacccctggtggatctgcccatcggcatcaacatcacccggtttcagaccctgcacagaagctacctgacacctggcgatagcagcagcggatggacagctggtgccgccgcttactatgtgggctacctgcagcctagaaccttcctgctgaagtacaacgagaacggcaccatcaccgacgccgtggattgtgctctggatcctctgagcgagacaaagtgcaccctgaagtccttcaccgtggaaaagggcatctaccagaccagcaacttccgggtgcagcccaccgaatccatcgtgcggttccccaatatcaccaatctgtgccccttcggcgaggtgttcaatgccaccagattcgcctctgtgtacgcctggaaccggaagcggatcagcaattgcgtggccgactactccgtgctgtacaactccgccagcttcagcaccttcaagtgctacggcgtgtcccctaccaagctgaacgacctgtgcttcacaaacgtgtacgccgacagcttcgtgatccggggagatgaagtgcggcagattgcccctggacagacaggcaatatcgccgactacaactacaagctgcccgacgacttcaccggctgtgtgattgcctggaacagcaacaacctggactccaaagtcggcggcaactacaattacctgtaccggctgttccggaagtccaatctgaagcccttcgagcgggacatctccaccgagatctatcaggccggcagcaccccttgtaacggcgtgaaaggcttcaactgctacttcccactgcagtcctacggctttcagcccacatatggcgtgggctatcagccctacagagtggtggtgctgagcttcgaactgctgcatgcccctgccacagtgtgcggccctaagaaaagcaccaatctcgtgaagaacaaatgcgtgaacttcaacttcaacggcctgaccggcaccggcgtgctgacagagagcaacaagaagttcctgccattccagcagtttggccgggatatcgccgataccacagacgccgttagagatccccagacactggaaatcctggacatcaccccttgcagcttcggcggagtgtctgtgatcacccctggcaccaacaccagcaatcaggtggcagtgctgtaccagggcgtgaactgtaccgaagtgcccgtggccattcacgccgatcagctgacacctacatggcgggtgtactccaccggcagcaatgtgtttcagaccagagccggctgtctgatcggagccgagcacgtgaacaatagctacgagtgcgacatccccatcggcgctggcatctgtgccagctaccagacacagacaaacagccccagacgggccagatctgtggccagccagagcatcattgcctacacaatgtctctgggcgtcgagaacagcgtggcctactccaacaactctatcgctatccccaccaacttcaccatcagcgtgaccacagagatcctgcctgtgtccatgaccaagaccagcgtggactgcaccatgtacatctgcggcgattccaccgagtgctccaacctgctgctgcagtacggcagcttctgcacccagctgaatagagccctgacagggatcgccgtggaacaggacaagaacacccaagaggtgttcgcccaagtgaagcagatctacaagacccctcctatcaaggacttcggcggcttcaatttcagccagattctgcccgatcctagcaagcccagcaagcggagcttcatcgaggacctgctgttcaacaaagtgacactggccgacgccggcttcatcaagcagtatggcgattgtctgggcgacattgccgccagggatctgatttgcgcccagaagtttaacggactgacagtgctgcctcctctgctgaccgatgagatgatcgcccagtacacatctgccctgctggccggcacaatcacaagcggctggacatttggagctggcgccgctctgcagatcccctttgctatgcagatggcctaccggttcaacggcatcggagtgacccagaatgtgctgtacgagaaccagaagctgatcgccaaccagttcaacagcgccatcggcaagatccaggacagcctgagcagcacagcaagcgccctgggaaagctgcaggacgtggtcaaccagaatgcccaggcactgaacaccctggtcaagcagctgtcctccaacttcggcgccatcagctctgtgctgaacgatatcctgagcagactggacaaggtggaagccgaggtgcagatcgacagactgatcaccggaaggctgcagtccctgcagacctacgttacccagcagctgatcagagccgccgagattagagcctctgccaatctggccgccaccaagatgtctgagtgtgtgctgggccagagcaagagagtggacttttgcggcaagggctaccacctgatgagcttccctcagtctgcccctcacggcgtggtgtttctgcacgtgacatacgtgcccgctcaagagaagaatttcaccaccgctccagccatctgccacgacggcaaagcccactttcctagagaaggcgtgttcgtgtccaacggcacccattggttcgtgacccagcggaacttctacgagccccagatcatcaccaccgacaacaccttcgtgtctggcaactgcgacgtcgtgatcggcattgtgaacaataccgtgtacgaccctctgcagcccgagctggacagcttcaaagaggaactggataagtactttaagaaccacacaagccccgacgtggacctgggcgatatcagcggaatcaatgccagcgtcgtgaacatccagaaagagatcgaccggctgaacgaggtggccaagaatctgaacgagagcctgatcgacctgcaagaactggggaagtacgagcagtacatcaagtggccctggtacatctggctgggctttatcgccggactgattgccatcgtgatggtcacaatcatgctgtgttgcatgaccagctgctgtagctgcctgaagggctgttgtagctgtggcagctgctgctga

SEQ ID NO: 54 - protein, 1251 aa, synthetic construct
  REGION 1..1251: note = Synthetic Construct
MFVFLVLLPLVSSQCVNFTTRTQLPPAYTNSFTRGVYYPDKVFRSSVLHSTQDLFLPFFSNVTWFHAIHVSGTNGTKRFANPVLPFNDGVYFASTEKSNIIRGWIFGTTLDSKTQSLLIVNNATNVVIKVCEFQFCNDPFLGVYYHKNNKSWMESEFRVYSSANNCTFEYVSQPFLMDLEGKQGNFKNLREFVFKNIDGYFKIYSKHTPINLVRGLPQGFSALEPLVDLPIGINITRFQTLHRSYLTPGDSSSGWTAGAAAYYVGYLQPRTFLLKYNENGTITDAVDCALDPLSETKCTLKSFTVEKGIYQTSNFRVQPTESIVRFPNITNLCPFGEVFNATRFASVYAWNRKRISNCVADYSVLYNSASFSTFKCYGVSPTKLNDLCFTNVYADSFVIRGDEVRQIAPGQTGNIADYNYKLPDDFTGCVIAWNSNNLDSKVGGNYNYLYRLFRKSNLKPFERDISTEIYQAGSTPCNGVKGFNCYFPLQSYGFQPTYGVGYQPYRVVVLSFELLHAPATVCGPKKSTNLVKNKCVNFNFNGLTGTGVLTESNKKFLPFQQFGRDIADTTDAVRDPQTLEILDITPCSFGGVSVITPGTNTSNQVAVLYQGVNCTEVPVAIHADQLTPTWRVYSTGSNVFQTRAGCLIGAEHVNNSYECDIPIGAGICASYQTQTNSPRRARSVASQSIIAYTMSLGVENSVAYSNNSIAIPTNFTISVTTEILPVSMTKTSVDCTMYICGDSTECSNLLLQYGSFCTQLNRALTGIAVEQDKNTQEVFAQVKQIYKTPPIKDFGGFNFSQILPDPSKPSKRSFIEDLLFNKVTLADAGFIKQYGDCLGDIAARDLICAQKFNGLTVLPPLLTDEMIAQYTSALLAGTITSGWTFGAGAALQIPFAMQMAYRFNGIGVTQNVLYENQKLIANQFNSAIGKIQDSLSSTASALGKLQDVVNQNAQALNTLVKQLSSNFGAISSVLNDILSRLDKVEAEVQIDRLITGRLQSLQTYVTQQLIRAAEIRASANLAATKMSECVLGQSKRVDFCGKGYHLMSFPQSAPHGVVFLHVTYVPAQEKNFTTAPAICHDGKAHFPREGVFVSNGTHWFVTQRNFYEPQIITTDNTFVSGNCDVVIGIVNNTVYDPLQPELDSFKEELDKYFKNHTSPDVDLGDISGINASVVNIQKEIDRLNEVAKNLNESLIDLQELGKYEQYIKWPWYIWLGFIAGLIAIVMVTIMLCCMTSCCSCLKGCCSCGSCC

SEQ ID NO: 55 - DNA, 3819 bp, synthetic construct
  misc_feature 1..3819: note = synthetic polynucleotide for Antigen_1_nCov_Spike_full_opt_h.sapiens_koz_SA_2P
  source 1..3819: mol_type = other DNA
  CDS 7..3819
gccaccatgttcgtgtttctggtgctgctgcctctggtgtccagccagtgtgtgaactttaccaccagaacacagctgcctccagcctacaccaacagctttaccagaggcgtgtactaccccgacaaggtgttcagatccagcgtgctgcactctacccaggacctgttcctgcctttcttcagcaacgtgacctggttccacgccatccacgtgtccggcaccaatggcaccaagagattcgccaaccccgtgctgcccttcaacgacggggtgtactttgccagcaccgagaagtccaacatcatcagaggctggatcttcggcaccacactggacagcaagacccagagcctgctgatcgtgaacaacgccaccaacgtggtcatcaaagtgtgcgagttccagttctgcaacgaccccttcctgggcgtctactaccacaagaacaacaagagctggatggaaagcgagttccgggtgtacagcagcgccaacaactgcaccttcgagtacgtgtcccagcctttcctgatggacctggaaggcaagcagggcaacttcaagaacctgcgcgagttcgtgttcaagaacatcgacggctacttcaagatctacagcaagcacacccctatcaacctcgtgcggggtctgcctcagggcttctctgctctggaacccctggtggatctgcccatcggcatcaacatcacccggtttcagaccctgcacagaagctacctgacacctggcgatagcagcagcggatggacagctggtgccgccgcttactatgtgggctacctgcagcctagaaccttcctgctgaagtacaacgagaacggcaccatcaccgacgccgtggattgtgctctggatcctctgagcgagacaaagtgcaccctgaagtccttcaccgtggaaaagggcatctaccagaccagcaacttccgggtgcagcccaccgaatccatcgtgcggttccccaatatcaccaatctgtgccccttcggcgaggtgttcaatgccaccagattcgcctctgtgtacgcctggaaccggaagcggatcagcaattgcgtggccgactactccgtgctgtacaactccgccagcttcagcaccttcaagtgctacggcgtgtcccctaccaagctgaacgacctgtgcttcacaaacgtgtacgccgacagcttcgtgatccggggagatgaagtgcggcagattgcccctggacagacaggcaatatcgccgactacaactacaagctgcccgacgacttcaccggctgtgtgattgcctggaacagcaacaacctggactccaaagtcggcggcaactacaattacctgtaccggctgttccggaagtccaatctgaagcccttcgagcgggacatctccaccgagatctatcaggccggcagcaccccttgtaacggcgtgaaaggcttcaactgctacttcccactgcagtcctacggctttcagcccacatatggcgtgggctatcagccctacagagtggtggtgctgagcttcgaactgctgcatgcccctgccacagtgtgcggccctaagaaaagcaccaatctcgtgaagaacaaatgcgtgaacttcaacttcaacggcctgaccggcaccggcgtgctgacagagagcaacaagaagttcctgccattccagcagtttggccgggatatcgccgataccacagacgccgttagagatccccagacactggaaatcctggacatcaccccttgcagcttcggcggagtgtctgtgatcacccctggcaccaacaccagcaatcaggtggcagtgctgtaccagggcgtgaactgtaccgaagtgcccgtggccattcacgccgatcagctgacacctacatggcgggtgtactccaccggcagcaatgtgtttcagaccagagccggctgtctgatcggagccgagcacgtgaacaatagctacgagtgcgacatccccatcggcgctggcatctgtgccagctaccagacacagacaaacagccccagacgggccagatctgtggccagccagagcatcattgcctacacaatgtctctgggcgtcgagaacagcgtggcctactccaacaactctatcgctatccccaccaacttcaccatcagcgtgaccacagagatcctgcctgtgtccatgaccaagaccagcgtggactgcaccatgtacatctgcggcgattccaccgagtgctccaacctgctgctgcagtacggcagcttctgcacccagctgaatagagccctgacagggatcgccgtggaacaggacaagaacacccaagaggtgttcgcccaagtgaagcagatctacaagacccctcctatcaaggacttcggcggcttcaatttcagccagattctgcccgatcctagcaagcccagcaagcggagcttcatcgaggacctgctgttcaacaaagtgacactggccgacgccggcttcatcaagcagtatggcgattgtctgggcgacattgccgccagggatctgatttgcgcccagaagtttaacggactgacagtgctgcctcctctgctgaccgatgagatgatcgcccagtacacatctgccctgctggccggcacaatcacaagcggctggacatttggagctggcgccgctctgcagatcccctttgctatgcagatggcctaccggttcaacggcatcggagtgacccagaatgtgctgtacgagaaccagaagctgatcgccaaccagttcaacagcgccatcggcaagatccaggacagcctgagcagcacagcaagcgccctgggaaagctgcaggacgtggtcaaccagaatgcccaggcactgaacaccctggtcaagcagctgtcctccaacttcggcgccatcagctctgtgctgaacgatatcctgagcagactggacccgccggaagccgaggtgcagatcgacagactgatcaccggaaggctgcagtccctgcagacctacgttacccagcagctgatcagagccgccgagattagagcctctgccaatctggccgccaccaagatgtctgagtgtgtgctgggccagagcaagagagtggacttttgcggcaagggctaccacctgatgagcttccctcagtctgcccctcacggcgtggtgtttctgcacgtgacatacgtgcccgctcaagagaagaatttcaccaccgctccagccatctgccacgacggcaaagcccactttcctagagaaggcgtgttcgtgtccaacggcacccattggttcgtgacccagcggaacttctacgagccccagatcatcaccaccgacaacaccttcgtgtctggcaactgcgacgtcgtgatcggcattgtgaacaataccgtgtacgaccctctgcagcccgagctggacagcttcaaagaggaactggataagtactttaagaaccacacaagccccgacgtggacctgggcgatatcagcggaatcaatgccagcgtcgtgaacatccagaaagagatcgaccggctgaacgaggtggccaagaatctgaacgagagcctgatcgacctgcaagaactggggaagtacgagcagtacatcaagtggccctggtacatctggctgggctttatcgccggactgattgccatcgtgatggtcacaatcatgctgtgttgcatgaccagctgctgtagctgcctgaagggctgttgtagctgtggcagctgctgcaagttcgacgaggacgattctgagcccgtgctgaagggcgtgaaactgcactacacctga

SEQ ID NO: 56 - protein, 1270 aa, synthetic construct
  REGION 1..1270: note = Synthetic Construct
MFVFLVLLPLVSSQCVNFTTRTQLPPAYTNSFTRGVYYPDKVFRSSVLHSTQDLFLPFFSNVTWFHAIHVSGTNGTKRFANPVLPFNDGVYFASTEKSNIIRGWIFGTTLDSKTQSLLIVNNATNVVIKVCEFQFCNDPFLGVYYHKNNKSWMESEFRVYSSANNCTFEYVSQPFLMDLEGKQGNFKNLREFVFKNIDGYFKIYSKHTPINLVRGLPQGFSALEPLVDLPIGINITRFQTLHRSYLTPGDSSSGWTAGAAAYYVGYLQPRTFLLKYNENGTITDAVDCALDPLSETKCTLKSFTVEKGIYQTSNFRVQPTESIVRFPNITNLCPFGEVFNATRFASVYAWNRKRISNCVADYSVLYNSASFSTFKCYGVSPTKLNDLCFTNVYADSFVIRGDEVRQIAPGQTGNIADYNYKLPDDFTGCVIAWNSNNLDSKVGGNYNYLYRLFRKSNLKPFERDISTEIYQAGSTPCNGVKGFNCYFPLQSYGFQPTYGVGYQPYRVVVLSFELLHAPATVCGPKKSTNLVKNKCVNFNFNGLTGTGVLTESNKKFLPFQQFGRDIADTTDAVRDPQTLEILDITPCSFGGVSVITPGTNTSNQVAVLYQGVNCTEVPVAIHADQLTPTWRVYSTGSNVFQTRAGCLIGAEHVNNSYECDIPIGAGICASYQTQTNSPRRARSVASQSIIAYTMSLGVENSVAYSNNSIAIPTNFTISVTTEILPVSMTKTSVDCTMYICGDSTECSNLLLQYGSFCTQLNRALTGIAVEQDKNTQEVFAQVKQIYKTPPIKDFGGFNFSQILPDPSKPSKRSFIEDLLFNKVTLADAGFIKQYGDCLGDIAARDLICAQKFNGLTVLPPLLTDEMIAQYTSALLAGTITSGWTFGAGAALQIPFAMQMAYRFNGIGVTQNVLYENQKLIANQFNSAIGKIQDSLSSTASALGKLQDVVNQNAQALNTLVKQLSSNFGAISSVLNDILSRLDPPEAEVQIDRLITGRLQSLQTYVTQQLIRAAEIRASANLAATKMSECVLGQSKRVDFCGKGYHLMSFPQSAPHGVVFLHVTYVPAQEKNFTTAPAICHDGKAHFPREGVFVSNGTHWFVTQRNFYEPQIITTDNTFVSGNCDVVIGIVNNTVYDPLQPELDSFKEELDKYFKNHTSPDVDLGDISGINASVVNIQKEIDRLNEVAKNLNESLIDLQELGKYEQYIKWPWYIWLGFIAGLIAIVMVTIMLCCMTSCCSCLKGCCSCGSCCKFDEDDSEPVLKGVKLHYT

SEQ ID NO: 57 - DNA, 3762 bp, synthetic construct
  misc_feature 1..3762: note = synthetic polynucleotide for Antigen_1_nCov_Spike_full_opt_h.sapiens_koz_SA_2P_delta_Cter
  source 1..3762: mol_type = other DNA
  CDS 7..3762
gccaccatgttcgtgtttctggtgctgctgcctctggtgtccagccagtgtgtgaactttaccaccagaacacagctgcctccagcctacaccaacagctttaccagaggcgtgtactaccccgacaaggtgttcagatccagcgtgctgcactctacccaggacctgttcctgcctttcttcagcaacgtgacctggttccacgccatccacgtgtccggcaccaatggcaccaagagattcgccaaccccgtgctgcccttcaacgacggggtgtactttgccagcaccgagaagtccaacatcatcagaggctggatcttcggcaccacactggacagcaagacccagagcctgctgatcgtgaacaacgccaccaacgtggtcatcaaagtgtgcgagttccagttctgcaacgaccccttcctgggcgtctactaccacaagaacaacaagagctggatggaaagcgagttccgggtgtacagcagcgccaacaactgcaccttcgagtacgtgtcccagcctttcctgatggacctggaaggcaagcagggcaacttcaagaacctgcgcgagttcgtgttcaagaacatcgacggctacttcaagatctacagcaagcacacccctatcaacctcgtgcggggtctgcctcagggcttctctgctctggaacccctggtggatctgcccatcggcatcaacatcacccggtttcagaccctgcacagaagctacctgacacctggcgatagcagcagcggatggacagctggtgccgccgcttactatgtgggctacctgcagcctagaaccttcctgctgaagtacaacgagaacggcaccatcaccgacgccgtggattgtgctctggatcctctgagcgagacaaagtgcaccctgaagtccttcaccgtggaaaagggcatctaccagaccagcaacttccgggtgcagcccaccgaatccatcgtgcggttccccaatatcaccaatctgtgccccttcggcgaggtgttcaatgccaccagattcgcctctgtgtacgcctggaaccggaagcggatcagcaattgcgtggccgactactccgtgctgtacaactccgccagcttcagcaccttcaagtgctacggcgtgtcccctaccaagctgaacgacctgtgcttcacaaacgtgtacgccgacagcttcgtgatccggggagatgaagtgcggcagattgcccctggacagacaggcaatatcgccgactacaactacaagctgcccgacgacttcaccggctgtgtgattgcctggaacagcaacaacctggactccaaagtcggcggcaactacaattacctgtaccggctgttccggaagtccaatctgaagcccttcgagcgggacatctccaccgagatctatcaggccggcagcaccccttgtaacggcgtgaaaggcttcaactgctacttcccactgcagtcctacggctttcagcccacatatggcgtgggctatcagccctacagagtggtggtgctgagcttcgaactgctgcatgcccctgccacagtgtgcggccctaagaaaagcaccaatctcgtgaagaacaaatgcgtgaacttcaacttcaacggcctgaccggcaccggcgtgctgacagagagcaacaagaagttcctgccattccagcagtttggccgggatatcgccgataccacagacgccgttagagatccccagacactggaaatcctggacatcaccccttgcagcttcggcggagtgtctgtgatcacccctggcaccaacaccagcaatcaggtggcagtgctgtaccagggcgtgaactgtaccgaagtgcccgtggccattcacgccgatcagctgacacctacatggcgggtgtactccaccggcagcaatgtgtttcagaccagagccggctgtctgatcggagccgagcacgtgaacaatagctacgagtgcgacatccccatcggcgctggcatctgtgccagctaccagacacagacaaacagccccagacgggccagatctgtggccagccagagcatcattgcctacacaatgtctctgggcgtcgagaacagcgtggcctactccaacaactctatcgctatccccaccaacttcaccatcagcgtgaccacagagatcctgcctgtgtccatgaccaagaccagcgtggactgcaccatgtacatctgcggcgattccaccgagtgctccaacctgctgctgcagtacggcagcttctgcacccagctgaatagagccctgacagggatcgccgtggaacaggacaagaacacccaagaggtgttcgcccaagtgaagcagatctacaagacccctcctatcaaggacttcggcggcttcaatttcagccagattctgcccgatcctagcaagcccagcaagcggagcttcatcgaggacctgctgttcaacaaagtgacactggccgacgccggcttcatcaagcagtatggcgattgtctgggcgacattgccgccagggatctgatttgcgcccagaagtttaacggactgacagtgctgcctcctctgctgaccgatgagatgatcgcccagtacacatctgccctgctggccggcacaatcacaagcggctggacatttggagctggcgccgctctgcagatcccctttgctatgcagatggcctaccggttcaacggcatcggagtgacccagaatgtgctgtacgagaaccagaagctgatcgccaaccagttcaacagcgccatcggcaagatccaggacagcctgagcagcacagcaagcgccctgggaaagctgcaggacgtggtcaaccagaatgcccaggcactgaacaccctggtcaagcagctgtcctccaacttcggcgccatcagctctgtgctgaacgatatcctgagcagactggacccgccggaagccgaggtgcagatcgacagactgatcaccggaaggctgcagtccctgcagacctacgttacccagcagctgatcagagccgccgagattagagcctctgccaatctggccgccaccaagatgtctgagtgtgtgctgggccagagcaagagagtggacttttgcggcaagggctaccacctgatgagcttccctcagtctgcccctcacggcgtggtgtttctgcacgtgacatacgtgcccgctcaagagaagaatttcaccaccgctccagccatctgccacgacggcaaagcccactttcctagagaaggcgtgttcgtgtccaacggcacccattggttcgtgacccagcggaacttctacgagccccagatcatcaccaccgacaacaccttcgtgtctggcaactgcgacgtcgtgatcggcattgtgaacaataccgtgtacgaccctctgcagcccgagctggacagcttcaaagaggaactggataagtactttaagaaccacacaagccccgacgtggacctgggcgatatcagcggaatcaatgccagcgtcgtgaacatccagaaagagatcgaccggctgaacgaggtggccaagaatctgaacgagagcctgatcgacctgcaagaactggggaagtacgagcagtacatcaagtggccctggtacatctggctgggctttatcgccggactgattgccatcgtgatggtcacaatcatgctgtgttgcatgaccagctgctgtagctgcctgaagggctgttgtagctgtggcagctgctgctga

SEQ ID NO: 58 - protein, 1251 aa, synthetic construct
  REGION 1..1251: note = Synthetic Construct
MFVFLVLLPLVSSQCVNFTTRTQLPPAYTNSFTRGVYYPDKVFRSSVLHSTQDLFLPFFSNVTWFHAIHVSGTNGTKRFANPVLPFNDGVYFASTEKSNIIRGWIFGTTLDSKTQSLLIVNNATNVVIKVCEFQFCNDPFLGVYYHKNNKSWMESEFRVYSSANNCTFEYVSQPFLMDLEGKQGNFKNLREFVFKNIDGYFKIYSKHTPINLVRGLPQGFSALEPLVDLPIGINITRFQTLHRSYLTPGDSSSGWTAGAAAYYVGYLQPRTFLLKYNENGTITDAVDCALDPLSETKCTLKSFTVEKGIYQTSNFRVQPTESIVRFPNITNLCPFGEVFNATRFASVYAWNRKRISNCVADYSVLYNSASFSTFKCYGVSPTKLNDLCFTNVYADSFVIRGDEVRQIAPGQTGNIADYNYKLPDDFTGCVIAWNSNNLDSKVGGNYNYLYRLFRKSNLKPFERDISTEIYQAGSTPCNGVKGFNCYFPLQSYGFQPTYGVGYQPYRVVVLSFELLHAPATVCGPKKSTNLVKNKCVNFNFNGLTGTGVLTESNKKFLPFQQFGRDIADTTDAVRDPQTLEILDITPCSFGGVSVITPGTNTSNQVAVLYQGVNCTEVPVAIHADQLTPTWRVYSTGSNVFQTRAGCLIGAEHVNNSYECDIPIGAGICASYQTQTNSPRRARSVASQSIIAYTMSLGVENSVAYSNNSIAIPTNFTISVTTEILPVSMTKTSVDCTMYICGDSTECSNLLLQYGSFCTQLNRALTGIAVEQDKNTQEVFAQVKQIYKTPPIKDFGGFNFSQILPDPSKPSKRSFIEDLLFNKVTLADAGFIKQYGDCLGDIAARDLICAQKFNGLTVLPPLLTDEMIAQYTSALLAGTITSGWTFGAGAALQIPFAMQMAYRFNGIGVTQNVLYENQKLIANQFNSAIGKIQDSLSSTASALGKLQDVVNQNAQALNTLVKQLSSNFGAISSVLNDILSRLDPPEAEVQIDRLITGRLQSLQTYVTQQLIRAAEIRASANLAATKMSECVLGQSKRVDFCGKGYHLMSFPQSAPHGVVFLHVTYVPAQEKNFTTAPAICHDGKAHFPREGVFVSNGTHWFVTQRNFYEPQIITTDNTFVSGNCDVVIGIVNNTVYDPLQPELDSFKEELDKYFKNHTSPDVDLGDISGINASVVNIQKEIDRLNEVAKNLNESLIDLQELGKYEQYIKWPWYIWLGFIAGLIAIVMVTIMLCCMTSCCSCLKGCCSCGSCC

SEQ ID NO: 59 - DNA, 3828 bp, synthetic construct
  misc_feature 1..3828: note = synthetic polynucleotide for Antigen_1_nCov_Spike_full_opt_h.sapiens_koz_Br
  source 1..3828: mol_type = other DNA
  CDS 7..3828
gccaccatgttcgtgtttctggtgctgctgcctctggtgtccagccagtgtgtgaactttaccaacagaacacagctgccttcagcctacaccaacagctttaccagaggcgtgtactaccccgacaaggtgttcagatccagcgtgctgcactctacccaggacctgttcctgcctttcttcagcaacgtgacctggttccacgccatccacgtgtccggcaccaatggcaccaagagattcgacaaccccgtgctgcccttcaacgacggggtgtactttgccagcaccgagaagtccaacatcatcagaggctggatcttcggcaccacactggacagcaagacccagagcctgctgatcgtgaacaacgccaccaacgtggtcatcaaagtgtgcgagttccagttctgcaactaccccttcctgggcgtctactaccacaagaacaacaagagctggatggaaagcgagttccgggtgtacagcagcgccaacaactgcaccttcgagtacgtgtcccagcctttcctgatggacctggaaggcaagcagggcaacttcaagaacctgagtgagttcgtgttcaagaacatcgacggctacttcaagatctacagcaagcacacccctatcaacctcgtgcgggatctgcctcagggcttctctgctctggaacccctggtggatctgcccatcggcatcaacatcacccggtttcagacactgctggccctgcacagaagctacctgacacctggcgatagcagcagcggatggacagctggtgccgccgcttactatgtgggctacctgcagcctagaaccttcctgctgaagtacaacgagaacggcaccatcaccgacgccgtggattgtgctctggatcctctgagcgagacaaagtgcaccctgaagtccttcaccgtggaaaagggcatctaccagaccagcaacttccgggtgcagcccaccgaatccatcgtgcggttccccaatatcaccaatctgtgccccttcggcgaggtgttcaatgccaccagattcgcctctgtgtacgcctggaaccggaagcggatcagcaattgcgtggccgactactccgtgctgtacaactccgccagcttcagcaccttcaagtgctacggcgtgtcccctaccaagctgaacgacctgtgcttcacaaacgtgtacgccgacagcttcgtgatccggggagatgaagtgcggcagattgcccctggacagacaggcacgatcgccgactacaactacaagctgcccgacgacttcaccggctgtgtgattgcctggaacagcaacaacctggactccaaagtcggcggcaactacaattacctgtaccggctgttccggaagtccaatctgaagcccttcgagcgggacatctccaccgagatctatcaggccggcagcaccccttgtaacggcgtgaaaggcttcaactgctacttcccactgcagtcctacggctttcagcccacatatggcgtgggctatcagccctacagagtggtggtgctgagcttcgaactgctgcatgcccctgccacagtgtgcggccctaagaaaagcaccaatctcgtgaagaacaaatgcgtgaacttcaacttcaacggcctgaccggcaccggcgtgctgacagagagcaacaagaagttcctgccattccagcagtttggccgggatatcgccgataccacagacgccgttagagatccccagacactggaaatcctggacatcaccccttgcagcttcggcggagtgtctgtgatcacccctggcaccaacaccagcaatcaggtggcagtgctgtaccagggcgtgaactgtaccgaagtgcccgtggccattcacgccgatcagctgacacctacatggcgggtgtactccaccggcagcaatgtgtttcagaccagagccggctgtctgatcggagccgagtacgtgaacaatagctacgagtgcgacatccccatcggcgctggcatctgtgccagctaccagacacagacaaacagccccagacgggccagatctgtggccagccagagcatcattgcctacacaatgtctctgggcgccgagaacagcgtggcctactccaacaactctatcgctatccccaccaacttcaccatcagcgtgaccacagagatcctgcctgtgtccatgaccaagaccagcgtggactgcaccatgtacatctgcggcgattccaccgagtgctccaacctgctgctgcagtacggcagcttctgcacccagctgaatagagccctgacagggatcgccgtggaacaggacaagaacacccaagaggtgttcgcccaagtgaagcagatctacaagacccctcctatcaaggacttcggcggcttcaatttcagccagattctgcccgatcctagcaagcccagcaagcggagcttcatcgaggacctgctgttcaacaaagtgacactggccgacgccggcttcatcaagcagtatggcgattgtctgggcgacattgccgccagggatctgatttgcgcccagaagtttaacggactgacagtgctgcctcctctgctgaccgatgagatgatcgcccagtacacatctgccctgctggccggcacaatcacaagcggctggacatttggagctggcgccgctctgcagatcccctttgctatgcagatggcctaccggttcaacggcatcggagtgacccagaatgtgctgtacgagaaccagaagctgatcgccaaccagttcaacagcgccatcggcaagatccaggacagcctgagcagcacagcaagcgccctgggaaagctgcaggacgtggtcaaccagaatgcccaggcactgaacaccctggtcaagcagctgtcctccaacttcggcgccatcagctctgtgctgaacgatatcctgagcagactggacaaggtggaagccgaggtgcagatcgacagactgatcaccggaaggctgcagtccctgcagacctacgttacccagcagctgatcagagccgccgagattagagcctctgccaatctggccgccatcaagatgtctgagtgtgtgctgggccagagcaagagagtggacttttgcggcaagggctaccacctgatgagcttccctcagtctgcccctcacggcgtggtgtttctgcacgtgacatacgtgcccgctcaagagaagaatttcaccaccgctccagccatctgccacgacggcaaagcccactttcctagagaaggcgtgttcgtgtccaacggcacccattggttcgtgacccagcggaacttctacgagccccagatcatcaccaccgacaacaccttcgtgtctggcaactgcgacgtcgtgatcggcattgtgaacaataccgtgtacgaccctctgcagcccgagctggacagcttcaaagaggaactggataagtactttaagaaccacacaagccccgacgtggacctgggcgatatcagcggaatcaatgccagcttcgtgaacatccagaaagagatcgaccggctgaacgaggtggccaagaatctgaacgagagcctgatcgacctgcaagaactggggaagtacgagcagtacatcaagtggccctggtacatctggctgggctttatcgccggactgattgccatcgtgatggtcacaatcatgctgtgttgcatgaccagctgctgtagctgcctgaagggctgttgtagctgtggcagctgctgcaagttcgacgaggacgattctgagcccgtgctgaagggcgtgaaactgcactacacctga

SEQ ID NO: 60 - protein, 1273 aa, synthetic construct
  REGION 1..1273: note = Synthetic Construct
MFVFLVLLPLVSSQCVNFTNRTQLPSAYTNSFTRGVYYPDKVFRSSVLHSTQDLFLPFFSNVTWFHAIHVSGTNGTKRFDNPVLPFNDGVYFASTEKSNIIRGWIFGTTLDSKTQSLLIVNNATNVVIKVCEFQFCNYPFLGVYYHKNNKSWMESEFRVYSSANNCTFEYVSQPFLMDLEGKQGNFKNLSEFVFKNIDGYFKIYSKHTPINLVRDLPQGFSALEPLVDLPIGINITRFQTLLALHRSYLTPGDSSSGWTAGAAAYYVGYLQPRTFLLKYNENGTITDAVDCALDPLSETKCTLKSFTVEKGIYQTSNFRVQPTESIVRFPNITNLCPFGEVFNATRFASVYAWNRKRISNCVADYSVLYNSASFSTFKCYGVSPTKLNDLCFTNVYADSFVIRGDEVRQIAPGQTGTIADYNYKLPDDFTGCVIAWNSNNLDSKVGGNYNYLYRLFRKSNLKPFERDISTEIYQAGSTPCNGVKGFNCYFPLQSYGFQPTYGVGYQPYRVVVLSFELLHAPATVCGPKKSTNLVKNKCVNFNFNGLTGTGVLTESNKKFLPFQQFGRDIADTTDAVRDPQTLEILDITPCSFGGVSVITPGTNTSNQVAVLYQGVNCTEVPVAIHADQLTPTWRVYSTGSNVFQTRAGCLIGAEYVNNSYECDIPIGAGICASYQTQTNSPRRARSVASQSIIAYTMSLGAENSVAYSNNSIAIPTNFTISVTTEILPVSMTKTSVDCTMYICGDSTECSNLLLQYGSFCTQLNRALTGIAVEQDKNTQEVFAQVKQIYKTPPIKDFGGFNFSQILPDPSKPSKRSFIEDLLFNKVTLADAGFIKQYGDCLGDIAARDLICAQKFNGLTVLPPLLTDEMIAQYTSALLAGTITSGWTFGAGAALQIPFAMQMAYRFNGIGVTQNVLYENQKLIANQFNSAIGKIQDSLSSTASALGKLQDVVNQNAQALNTLVKQLSSNFGAISSVLNDILSRLDKVEAEVQIDRLITGRLQSLQTYVTQQLIRAAEIRASANLAAIKMSECVLGQSKRVDFCGKGYHLMSFPQSAPHGVVFLHVTYVPAQEKNFTTAPAICHDGKAHFPREGVFVSNGTHWFVTQRNFYEPQIITTDNTFVSGNCDVVIGIVNNTVYDPLQPELDSFKEELDKYFKNHTSPDVDLGDISGINASFVNIQKEIDRLNEVAKNLNESLIDLQELGKYEQYIKWPWYIWLGFIAGLIAIVMVTIMLCCMTSCCSCLKGCCSCGSCCKFDEDDSEPVLKGVKLHYT

SEQ ID NO: 61 - DNA, 3771 bp, synthetic construct
  misc_feature 1..3771: note = synthetic polynucleotide for Antigen_1_nCov_Spike_full_opt_h.sapiens_koz_Br_delta_Cter
  source 1..3771: mol_type = other DNA
  CDS 7..3771
gccaccatgttcgtgtttctggtgctgctgcctctggtgtccagccagtgtgtgaactttaccaacagaacacagctgccttcagcctacaccaacagctttaccagaggcgtgtactaccccgacaaggtgttcagatccagcgtgctgcactctacccaggacctgttcctgcctttcttcagcaacgtgacctggttccacgccatccacgtgtccggcaccaatggcaccaagagattcgacaaccccgtgctgcccttcaacgacggggtgtactttgccagcaccgagaagtccaacatcatcagaggctggatcttcggcaccacactggacagcaagacccagagcctgctgatcgtgaacaacgccaccaacgtggtcatcaaagtgtgcgagttccagttctgcaactaccccttcctgggcgtctactaccacaagaacaacaagagctggatggaaagcgagttccgggtgtacagcagcgccaacaactgcaccttcgagtacgtgtcccagcctttcctgatggacctggaaggcaagcagggcaacttcaagaacctgagtgagttcgtgttcaagaacatcgacggctacttcaagatctacagcaagcacacccctatcaacctcgtgcgggatctgcctcagggcttctctgctctggaacccctggtggatctgcccatcggcatcaacatcacccggtttcagacactgctggccctgcacagaagctacctgacacctggcgatagcagcagcggatggacagctggtgccgccgcttactatgtgggctacctgcagcctagaaccttcctgctgaagtacaacgagaacggcaccatcaccgacgccgtggattgtgctctggatcctctgagcgagacaaagtgcaccctgaagtccttcaccgtggaaaagggcatctaccagaccagcaacttccgggtgcagcccaccgaatccatcgtgcggttccccaatatcaccaatctgtgccccttcggcgaggtgttcaatgccaccagattcgcctctgtgtacgcctggaaccggaagcggatcagcaattgcgtggccgactactccgtgctgtacaactccgccagcttcagcaccttcaagtgctacggcgtgtcccctaccaagctgaacgacctgtgcttcacaaacgtgtacgccgacagcttcgtgatccggggagatgaagtgcggcagattgcccctggacagacaggcacgatcgccgactacaactacaagctgcccgacgacttcaccggctgtgtgattgcctggaacagcaacaacctggactccaaagtcggcggcaactacaattacctgtaccggctgttccggaagtccaatctgaagcccttcgagcgggacatctccaccgagatctatcaggccggcagcaccccttgtaacggcgtgaaaggcttcaactgctacttcccactgcagtcctacggctttcagcccacatatggcgtgggctatcagccctacagagtggtggtgctgagcttcgaactgctgcatgcccctgccacagtgtgcggccctaagaaaagcaccaatctcgtgaagaacaaatgcgtgaacttcaacttcaacggcctgaccggcaccggcgtgctgacagagagcaacaagaagttcctgccattccagcagtttggccgggatatcgccgataccacagacgccgttagagatccccagacactggaaatcctggacatcaccccttgcagcttcggcggagtgtctgtgatcacccctggcaccaacaccagcaatcaggtggcagtgctgtaccagggcgtgaactgtaccgaagtgcccgtggccattcacgccgatcagctgacacctacatggcgggtgtactccaccggcagcaatgtgtttcagaccagagccggctgtctgatcggagccgagtacgtgaacaatagctacgagtgcgacatccccatcggcgctggcatctgtgccagctaccagacacagacaaacagccccagacgggccagatctgtggccagccagagcatcattgcctacacaatgtctctgggcgccgagaacagcgtggcctactccaacaactctatcgctatccccaccaacttcaccatcagcgtgaccacagagatcctgcctgtgtccatgaccaagaccagcgtggactgcaccatgtacatctgcggcgattccaccgagtgctccaacctgctgctgcagtacggcagcttctgcacccagctgaatagagccctgacagggatcgccgtggaacaggacaagaacacccaagaggtgttcgcccaagtgaagcagatctacaagacccctcctatcaaggacttcggcggcttcaatttcagccagattctgcccgatcctagcaagcccagcaagcggagcttcatcgaggacctgctgttcaacaaagtgacactggccgacgccggcttcatcaagcagtatggcgattgtctgggcgacattgccgccagggatctgatttgcgcccagaagtttaacggactgacagtgctgcctcctctgctgaccgatgagatgatcgcccagtacacatctgccctgctggccggcacaatcacaagcggctggacatttggagctggcgccgctctgcagatcccctttgctatgcagatggcctaccggttcaacggcatcggagtgacccagaatgtgctgtacgagaaccagaagctgatcgccaaccagttcaacagcgccatcggcaagatccaggacagcctgagcagcacagcaagcgccctgggaaagctgcaggacgtggtcaaccagaatgcccaggcactgaacaccctggtcaagcagctgtcctccaacttcggcgccatcagctctgtgctgaacgatatcctgagcagactggacaaggtggaagccgaggtgcagatcgacagactgatcaccggaaggctgcagtccctgcagacctacgttacccagcagctgatcagagccgccgagattagagcctctgccaatctggccgccatcaagatgtctgagtgtgtgctgggccagagcaagagagtggacttttgcggcaagggctaccacctgatgagcttccctcagtctgcccctcacggcgtggtgtttctgcacgtgacatacgtgcccgctcaagagaagaatttcaccaccgctccagccatctgccacgacggcaaagcccactttcctagagaaggcgtgttcgtgtccaacggcacccattggttcgtgacccagcggaacttctacgagccccagatcatcaccaccgacaacaccttcgtgtctggcaactgcgacgtcgtgatcggcattgtgaacaataccgtgtacgaccctctgcagcccgagctggacagcttcaaagaggaactggataagtactttaagaaccacacaagccccgacgtggacctgggcgatatcagcggaatcaatgccagcttcgtgaacatccagaaagagatcgaccggctgaacgaggtggccaagaatctgaacgagagcctgatcgacctgcaagaactggggaagtacgagcagtacatcaagtggccctggtacatctggctgggctttatcgccggactgattgccatcgtgatggtcacaatcatgctgtgttgcatgaccagctgctgtagctgcctgaagggctgttgtagctgtggcagctgctgctga

SEQ ID NO: 62 - protein, 1254 aa, synthetic construct
  REGION 1..1254: note = Synthetic Construct
MFVFLVLLPLVSSQCVNFTNRTQLPSAYTNSFTRGVYYPDKVFRSSVLHSTQDLFLPFFSNVTWFHAIHVSGTNGTKRFDNPVLPFNDGVYFASTEKSNIIRGWIFGTTLDSKTQSLLIVNNATNVVIKVCEFQFCNYPFLGVYYHKNNKSWMESEFRVYSSANNCTFEYVSQPFLMDLEGKQGNFKNLSEFVFKNIDGYFKIYSKHTPINLVRDLPQGFSALEPLVDLPIGINITRFQTLLALHRSYLTPGDSSSGWTAGAAAYYVGYLQPRTFLLKYNENGTITDAVDCALDPLSETKCTLKSFTVEKGIYQTSNFRVQPTESIVRFPNITNLCPFGEVFNATRFASVYAWNRKRISNCVADYSVLYNSASFSTFKCYGVSPTKLNDLCFTNVYADSFVIRGDEVRQIAPGQTGTIADYNYKLPDDFTGCVIAWNSNNLDSKVGGNYNYLYRLFRKSNLKPFERDISTEIYQAGSTPCNGVKGFNCYFPLQSYGFQPTYGVGYQPYRVVVLSFELLHAPATVCGPKKSTNLVKNKCVNFNFNGLTGTGVLTESNKKFLPFQQFGRDIADTTDAVRDPQTLEILDITPCSFGGVSVITPGTNTSNQVAVLYQGVNCTEVPVAIHADQLTPTWRVYSTGSNVFQTRAGCLIGAEYVNNSYECDIPIGAGICASYQTQTNSPRRARSVASQSIIAYTMSLGAENSVAYSNNSIAIPTNFTISVTTEILPVSMTKTSVDCTMYICGDSTECSNLLLQYGSFCTQLNRALTGIAVEQDKNTQEVFAQVKQIYKTPPIKDFGGFNFSQILPDPSKPSKRSFIEDLLFNKVTLADAGFIKQYGDCLGDIAARDLICAQKFNGLTVLPPLLTDEMIAQYTSALLAGTITSGWTFGAGAALQIPFAMQMAYRFNGIGVTQNVLYENQKLIANQFNSAIGKIQDSLSSTASALGKLQDVVNQNAQALNTLVKQLSSNFGAISSVLNDILSRLDKVEAEVQIDRLITGRLQSLQTYVTQQLIRAAEIRASANLAAIKMSECVLGQSKRVDFCGKGYHLMSFPQSAPHGVVFLHVTYVPAQEKNFTTAPAICHDGKAHFPREGVFVSNGTHWFVTQRNFYEPQIITTDNTFVSGNCDVVIGIVNNTVYDPLQPELDSFKEELDKYFKNHTSPDVDLGDISGINASFVNIQKEIDRLNEVAKNLNESLIDLQELGKYEQYIKWPWYIWLGFIAGLIAIVMVTIMLCCMTSCCSCLKGCCSCGSCC

SEQ ID NO: 63 - DNA, 3828 bp, synthetic construct
  misc_feature 1..3828: note = synthetic polynucleotide for Antigen_1_nCov_Spike_full_opt_h.sapiens_koz_Br_2P
  source 1..3828: mol_type = other DNA
  CDS 7..3828
gccaccatgttcgtgtttctggtgctgctgcctctggtgtccagccagtgtgtgaactttaccaacagaacacagctgccttcagcctacaccaacagctttaccagaggcgtgtactaccccgacaaggtgttcagatccagcgtgctgcactctacccaggacctgttcctgcctttcttcagcaacgtgacctggttccacgccatccacgtgtccggcaccaatggcaccaagagattcgacaaccccgtgctgcccttcaacgacggggtgtactttgccagcaccgagaagtccaacatcatcagaggctggatcttcggcaccacactggacagcaagacccagagcctgctgatcgtgaacaacgccaccaacgtggtcatcaaagtgtgcgagttccagttctgcaactaccccttcctgggcgtctactaccacaagaacaacaagagctggatggaaagcgagttccgggtgtacagcagcgccaacaactgcaccttcgagtacgtgtcccagcctttcctgatggacctggaaggcaagcagggcaacttcaagaacctgagtgagttcgtgttcaagaacatcgacggctacttcaagatctacagcaagcacacccctatcaacctcgtgcgggatctgcctcagggcttctctgctctggaacccctggtggatctgcccatcggcatcaacatcacccggtttcagacactgctggccctgcacagaagctacctgacacctggcgatagcagcagcggatggacagctggtgccgccgcttactatgtgggctacctgcagcctagaaccttcctgctgaagtacaacgagaacggcaccatcaccgacgccgtggattgtgctctggatcctctgagcgagacaaagtgcaccctgaagtccttcaccgtggaaaagggcatctaccagaccagcaacttccgggtgcagcccaccgaatccatcgtgcggttccccaatatcaccaatctgtgccccttcggcgaggtgttcaatgccaccagattcgcctctgtgtacgcctggaaccggaagcggatcagcaattgcgtggccgactactccgtgctgtacaactccgccagcttcagcaccttcaagtgctacggcgtgtcccctaccaagctgaacgacctgtgcttcacaaacgtgtacgccgacagcttcgtgatccggggagatgaagtgcggcagattgcccctggacagacaggcacgatcgccgactacaactacaagctgcccgacgacttcaccggctgtgtgattgcctggaacagcaacaacctggactccaaagtcggcggcaactacaattacctgtaccggctgttccggaagtccaatctgaagcccttcgagcgggacatctccaccgagatctatcaggccggcagcaccccttgtaacggcgtgaaaggcttcaactgctacttcccactgcagtcctacggctttcagcccacatatggcgtgggctatcagccctacagagtggtggtgctgagcttcgaactgctgcatgcccctgccacagtgtgcggccctaagaaaagcaccaatctcgtgaagaacaaatgcgtgaacttcaacttcaacggcctgaccggcaccggcgtgctgacagagagcaacaagaagttcctgccattccagcagtttggccgggatatcgccgataccacagacgccgttagagatccccagacactggaaatcctggacatcaccccttgcagcttcggcggagtgtctgtgatcacccctggcaccaacaccagcaatcaggtggcagtgctgtaccagggcgtgaactgtaccgaagtgcccgtggccattcacgccgatcagctgacacctacatggcgggtgtactccaccggcagcaatgtgtttcagaccagagccggctgtctgatcggagccgagtacgtgaacaatagctacgagtgcgacatccccatcggcgctggcatctgtgccagctaccagacacagacaaacagccccagacgggccagatctgtggccagccagagcatcattgcctacacaatgtctctgggcgccgagaacagcgtggcctactccaacaactctatcgctatccccaccaacttcaccatcagcgtgaccacagagatcctgcctgtgtccatgaccaagaccagcgtggactgcaccatgtacatctgcggcgattccaccgagtgctccaacctgctgctgcagtacggcagcttctgcacccagctgaatagagccctgacagggatcgccgtggaacaggacaagaacacccaagaggtgttcgcccaagtgaagcagatctacaagacccctcctatcaaggacttcggcggcttcaatttcagccagattctgcccgatcctagcaagcccagcaagcggagcttcatcgaggacctgctgttcaacaaagtgacactggccgacgccggcttcatcaagcagtatggcgattgtctgggcgacattgccgccagggatctgatttgcgcccagaagtttaacggactgacagtgctgcctcctctgctgaccgatgagatgatcgcccagtacacatctgccctgctggccggcacaatcacaagcggctggacatttggagctggcgccgctctgcagatcccctttgctatgcagatggcctaccggttcaacggcatcggagtgacccagaatgtgctgtacgagaaccagaagctgatcgccaaccagttcaacagcgccatcggcaagatccaggacagcctgagcagcacagcaagcgccctgggaaagctgcaggacgtggtcaaccagaatgcccaggcactgaacaccctggtcaagcagctgtcctccaacttcggcgccatcagctctgtgctgaacgatatcctgagcagactggacccgccggaagccgaggtgcagatcgacagactgatcaccggaaggctgcagtccctgcagacctacgttacccagcagctgatcagagccgccgagattagagcctctgccaatctggccgccatcaagatgtctgagtgtgtgctgggccagagcaagagagtggacttttgcggcaagggctaccacctgatgagcttccctcagtctgcccctcacggcgtggtgtttctgcacgtgacatacgtgcccgctcaagagaagaatttcaccaccgctccagccatctgccacgacggcaaagcccactttcctagagaaggcgtgttcgtgtccaacggcacccattggttcgtgacccagcggaacttctacgagccccagatcatcaccaccgacaacaccttcgtgtctggcaactgcgacgtcgtgatcggcattgtgaacaataccgtgtacgaccctctgcagcccgagctggacagcttcaaagaggaactggataagtactttaagaaccacacaagccccgacgtggacctgggcgatatcagcggaatcaatgccagcttcgtgaacatccagaaagagatcgaccggctgaacgaggtggccaagaatctgaacgagagcctgatcgacctgcaagaactggggaagtacgagcagtacatcaagtggccctggtacatctggctgggctttatcgccggactgattgccatcgtgatggtcacaatcatgctgtgttgcatgaccagctgctgtagctgcctgaagggctgttgtagctgtggcagctgctgcaagttcgacgaggacgattctgagcccgtgctgaagggcgtgaaactgcactacacctga

SEQ ID NO: 64 - protein, 1273 aa, synthetic construct
  REGION 1..1273: note = Synthetic Construct
MFVFLVLLPLVSSQCVNFTNRTQLPSAYTNSFTRGVYYPDKVFRSSVLHSTQDLFLPFFSNVTWFHAIHVSGTNGTKRFDNPVLPFNDGVYFASTEKSNIIRGWIFGTTLDSKTQSLLIVNNATNVVIKVCEFQFCNYPFLGVYYHKNNKSWMESEFRVYSSANNCTFEYVSQPFLMDLEGKQGNFKNLSEFVFKNIDGYFKIYSKHTPINLVRDLPQGFSALEPLVDLPIGINITRFQTLLALHRSYLTPGDSSSGWTAGAAAYYVGYLQPRTFLLKYNENGTITDAVDCALDPLSETKCTLKSFTVEKGIYQTSNFRVQPTESIVRFPNITNLCPFGEVFNATRFASVYAWNRKRISNCVADYSVLYNSASFSTFKCYGVSPTKLNDLCFTNVYADSFVIRGDEVRQIAPGQTGTIADYNYKLPDDFTGCVIAWNSNNLDSKVGGNYNYLYRLFRKSNLKPFERDISTEIYQAGSTPCNGVKGFNCYFPLQSYGFQPTYGVGYQPYRVVVLSFELLHAPATVCGPKKSTNLVKNKCVNFNFNGLTGTGVLTESNKKFLPFQQFGRDIADTTDAVRDPQTLEILDITPCSFGGVSVITPGTNTSNQVAVLYQGVNCTEVPVAIHADQLTPTWRVYSTGSNVFQTRAGCLIGAEYVNNSYECDIPIGAGICASYQTQTNSPRRARSVASQSIIAYTMSLGAENSVAYSNNSIAIPTNFTISVTTEILPVSMTKTSVDCTMYICGDSTECSNLLLQYGSFCTQLNRALTGIAVEQDKNTQEVFAQVKQIYKTPPIKDFGGFNFSQILPDPSKPSKRSFIEDLLFNKVTLADAGFIKQYGDCLGDIAARDLICAQKFNGLTVLPPLLTDEMIAQYTSALLAGTITSGWTFGAGAALQIPFAMQMAYRFNGIGVTQNVLYENQKLIANQFNSAIGKIQDSLSSTASALGKLQDVVNQNAQALNTLVKQLSSNFGAISSVLNDILSRLDPPEAEVQIDRLITGRLQSLQTYVTQQLIRAAEIRASANLAAIKMSECVLGQSKRVDFCGKGYHLMSFPQSAPHGVVFLHVTYVPAQEKNFTTAPAICHDGKAHFPREGVFVSNGTHWFVTQRNFYEPQIITTDNTFVSGNCDVVIGIVNNTVYDPLQPELDSFKEELDKYFKNHTSPDVDLGDISGINASFVNIQKEIDRLNEVAKNLNESLIDLQELGKYEQYIKWPWYIWLGFIAGLIAIVMVTIMLCCMTSCCSCLKGCCSCGSCCKFDEDDSEPVLKGVKLHYT

SEQ ID NO: 65 - DNA, 3771 bp, synthetic construct
  misc_feature 1..3771: note = synthetic polynucleotide for Antigen_1_nCov_Spike_full_opt_h.sapiens_koz_Br_2P_delta_Cter
  source 1..3771: mol_type = other DNA
  CDS 7..3771
gccaccatgttcgtgtttctggtgctgctgcctctggtgtccagccagtgtgtgaactttaccaacagaacacagctgccttcagcctacaccaacagctttaccagaggcgtgtactaccccgacaaggtgttcagatccagcgtgctgcactctacccaggacctgttcctgcctttcttcagcaacgtgacctggttccacgccatccacgtgtccggcaccaatggcaccaagagattcgacaaccccgtgctgcccttcaacgacggggtgtactttgccagcaccgagaagtccaacatcatcagaggctggatcttcggcaccacactggacagcaagacccagagcctgctgatcgtgaacaacgccaccaacgtggtcatcaaagtgtgcgagttccagttctgcaactaccccttcctgggcgtctactaccacaagaacaacaagagctggatggaaagcgagttccgggtgtacagcagcgccaacaactgcaccttcgagtacgtgtcccagcctttcctgatggacctggaaggcaagcagggcaacttcaagaacctgagtgagttcgtgttcaagaacatcgacggctacttcaagatctacagcaagcacacccctatcaacctcgtgcgggatctgcctcagggcttctctgctctggaacccctggtggatctgcccatcggcatcaacatcacccggtttcagacactgctggccctgcacagaagctacctgacacctggcgatagcagcagcggatggacagctggtgccgccgcttactatgtgggctacctgcagcctagaaccttcctgctgaagtacaacgagaacggcaccatcaccgacgccgtggattgtgctctggatcctctgagcgagacaaagtgcaccctgaagtccttcaccgtggaaaagggcatctaccagaccagcaacttccgggtgcagcccaccgaatccatcgtgcggttccccaatatcaccaatctgtgccccttcggcgaggtgttcaatgccaccagattcgcctctgtgtacgcctggaaccggaagcggatcagcaattgcgtggccgactactccgtgctgtacaactccgccagcttcagcaccttcaagtgctacggcgtgtcccctaccaagctgaacgacctgtgcttcacaaacgtgtacgccgacagcttcgtgatccggggagatgaagtgcggcagattgcccctggacagacaggcacgatcgccgactacaactacaagctgcccgacgacttcaccggctgtgtgattgcctggaacagcaacaacctggactccaaagtcggcggcaactacaattacctgtaccggctgttccggaagtccaatctgaagcccttcgagcgggacatctccaccgagatctatcaggccggcagcaccccttgtaacggcgtgaaaggcttcaactgctacttcccactgcagtcctacggctttcagcccacatatggcgtgggctatcagccctacagagtggtggtgctgagcttcgaactgctgcatgcccctgccacagtgtgcggccctaagaaaagcaccaatctcgtgaagaacaaatgcgtgaacttcaacttcaacggcctgaccggcaccggcgtgctgacagagagcaacaagaagttcctgccattccagcagtttggccgggatatcgccgataccacagacgccgttagagatccccagacactggaaatcctggacatcaccccttgcagcttcggcggagtgtctgtgatcacccctggcaccaacaccagcaatcaggtggcagtgctgtaccagggcgtgaactgtaccgaagtgcccgtggccattcacgccgatcagctgacacctacatggcgggtgtactccaccggcagcaatgtgtttcagaccagagccggctgtctgatcggagccgagtacgtgaacaatagctacgagtgcgacatccccatcggcgctggcatctgtgccagctaccagacacagacaaacagccccagacgggccagatctgtggccagccagagcatcattgcctacacaatgtctctgggcgccgagaacagcgtggcctactccaacaactctatcgctatccccaccaacttcaccatcagcgtgaccacagagatcctgcctgtgtccatgaccaagaccagcgtggactgcaccatgtacatctgcggcgattccaccgagtgctccaacctgctgctgcagtacggcagcttctgcacccagctgaatagagccctgacagggatcgccgtggaacaggacaagaacacccaagaggtgttcgcccaagtgaagcagatctacaagacccctcctatcaaggacttcggcggcttcaatttcagccagattctgcccgatcctagcaagcccagcaagcggagcttcatcgaggacctgctgttcaacaaagtgacactggccgacgccggcttcatcaagcagtatggcgattgtctgggcgacattgccgccagggatctgatttgcgcccagaagtttaacggactgacagtgctgcctcctctgctgaccgatgagatgatcgcccagtacacatctgccctgctggccggcacaatcacaagcggctggacatttggagctggcgccgctctgcagatcccctttgctatgcagatggcctaccggttcaacggcatcggagtgacccagaatgtgctgtacgagaaccagaagctgatcgccaaccagttcaacagcgccatcggcaagatccaggacagcctgagcagcacagcaagcgccctgggaaagctgcaggacgtggtcaaccagaatgcccaggcactgaacaccctggtcaagcagctgtcctccaacttcggcgccatcagctctgtgctgaacgatatcctgagcagactggacccgccggaagccgaggtgcagatcgacagactgatcaccggaaggctgcagtccctgcagacctacgttacccagcagctgatcagagccgccgagattagagcctctgccaatctggccgccatcaagatgtctgagtgtgtgctgggccagagcaagagagtggacttttgcggcaagggctaccacctgatgagcttccctcagtctgcccctcacggcgtggtgtttctgcacgtgacatacgtgcccgctcaagagaagaatttcaccaccgctccagccatctgccacgacggcaaagcccactttcctagagaaggcgtgttcgtgtccaacggcacccattggttcgtgacccagcggaacttctacgagccccagatcatcaccaccgacaacaccttcgtgtctggcaactgcgacgtcgtgatcggcattgtgaacaataccgtgtacgaccctctgcagcccgagctggacagcttcaaagaggaactggataagtactttaagaaccacacaagccccgacgtggacctgggcgatatcagcggaatcaatgccagcttcgtgaacatccagaaagagatcgaccggctgaacgaggtggccaagaatctgaacgagagcctgatcgacctgcaagaactggggaagtacgagcagtacatcaagtggccctggtacatctggctgggctttatcgccggactgattgccatcgtgatggtcacaatcatgctgtgttgcatgaccagctgctgtagctgcctgaagggctgttgtagctgtggcagctgctgctga

SEQ ID NO: 66 - protein, 1254 aa, synthetic construct
  REGION 1..1254: note = Synthetic Construct
MFVFLVLLPLVSSQCVNFTNRTQLPSAYTNSFTRGVYYPDKVFRSSVLHSTQDLFLPFFSNVTWFHAIHVSGTNGTKRFDNPVLPFNDGVYFASTEKSNIIRGWIFGTTLDSKTQSLLIVNNATNVVIKVCEFQFCNYPFLGVYYHKNNKSWMESEFRVYSSANNCTFEYVSQPFLMDLEGKQGNFKNLSEFVFKNIDGYFKIYSKHTPINLVRDLPQGFSALEPLVDLPIGINITRFQTLLALHRSYLTPGDSSSGWTAGAAAYYVGYLQPRTFLLKYNENGTITDAVDCALDPLSETKCTLKSFTVEKGIYQTSNFRVQPTESIVRFPNITNLCPFGEVFNATRFASVYAWNRKRISNCVADYSVLYNSASFSTFKCYGVSPTKLNDLCFTNVYADSFVIRGDEVRQIAPGQTGTIADYNYKLPDDFTGCVIAWNSNNLDSKVGGNYNYLYRLFRKSNLKPFERDISTEIYQAGSTPCNGVKGFNCYFPLQSYGFQPTYGVGYQPYRVVVLSFELLHAPATVCGPKKSTNLVKNKCVNFNFNGLTGTGVLTESNKKFLPFQQFGRDIADTTDAVRDPQTLEILDITPCSFGGVSVITPGTNTSNQVAVLYQGVNCTEVPVAIHADQLTPTWRVYSTGSNVFQTRAGCLIGAEYVNNSYECDIPIGAGICASYQTQTNSPRRARSVASQSIIAYTMSLGAENSVAYSNNSIAIPTNFTISVTTEILPVSMTKTSVDCTMYICGDSTECSNLLLQYGSFCTQLNRALTGIAVEQDKNTQEVFAQVKQIYKTPPIKDFGGFNFSQILPDPSKPSKRSFIEDLLFNKVTLADAGFIKQYGDCLGDIAARDLICAQKFNGLTVLPPLLTDEMIAQYTSALLAGTITSGWTFGAGAALQIPFAMQMAYRFNGIGVTQNVLYENQKLIANQFNSAIGKIQDSLSSTASALGKLQDVVNQNAQALNTLVKQLSSNFGAISSVLNDILSRLDPPEAEVQIDRLITGRLQSLQTYVTQQLIRAAEIRASANLAAIKMSECVLGQSKRVDFCGKGYHLMSFPQSAPHGVVFLHVTYVPAQEKNFTTAPAICHDGKAHFPREGVFVSNGTHWFVTQRNFYEPQIITTDNTFVSGNCDVVIGIVNNTVYDPLQPELDSFKEELDKYFKNHTSPDVDLGDISGINASFVNIQKEIDRLNEVAKNLNESLIDLQELGKYEQYIKWPWYIWLGFIAGLIAIVMVTIMLCCMTSCCSCLKGCCSCGSCC